European Patent Specification EP 3 702 367 B1, published May 15, 2024. Title: NOVEL PD-L1 BINDING POLYPEPTIDES FOR IMAGING. Applicant: BRISTOL-MYERS SQUIBB COMPANY. Application PCT/US2015/062485. The sequence listing filed with the application follows.

SEQUENCE LISTING (685 sequences)

SEQ ID NO: 1 - protein, 94 aa, Homo sapiens
  misc_feature: Full length wild-type human 10Fn3 domain
VSDVPRDLEVVAATPTSLLISWDAPAVTVRYYRITYGETGGNSPVQEFTVPGSKSTATISGLKPGVDYTITVYAVTGRGDSPASSKPISINYRT

SEQ ID NO: 2 - protein, 86 aa, Homo sapiens
  misc_feature: Core wild-type human 10Fn3 domain
EVVAATPTSLLISWDAPAVTVRYYRITYGETGGNSPVQEFTVPGSKSTATISGLKPGVDYTITVYAVTGRGDSPASSKPISINYRT

SEQ ID NO: 3 - protein, 128 aa, Artificial Sequence
  Synthetic: Core 10Fn3-based scaffold with variable AB, BC, CD, DE, EF, and FG loops
  misc_feature (6)..(20): Xaa can be any naturally occurring amino acid; at least one amino acid must be present, the rest may be present or absent
  misc_feature (26)..(40): Xaa can be any naturally occurring amino acid; at least two amino acids must be present, the rest may be present or absent
  misc_feature (46)..(60): Xaa can be any naturally occurring amino acid; at least two amino acids must be present, the rest may be present or absent
  misc_feature (64)..(78): Xaa can be any naturally occurring amino acid; at least two amino acids must be present, the rest may be present or absent
  misc_feature (85)..(99): Xaa can be any naturally occurring amino acid; at least two amino acids must be present, the rest may be present or absent
  misc_feature (107)..(121): Xaa can be any naturally occurring amino acid; at least two amino acids must be present, the rest may be present or absent
EVVAAXXXXXXXXXXXXXXXLLISWXXXXXXXXXXXXXXXYRITYXXXXXXXXXXXXXXXFTVXXXXXXXXXXXXXXXATISGLXXXXXXXXXXXXXXXYTITVYAXXXXXXXXXXXXXXXISINYRT

SEQ ID NO: 4 - protein, 103 aa, Artificial Sequence
  Synthetic: Core 10Fn3-based scaffold with variable BC, DE, and FG loops
  misc_feature (15)..(29): Xaa can be any naturally occurring amino acid; at least two amino acids must be present, the rest may be present or absent
  misc_feature (49)..(63): Xaa can be any naturally occurring amino acid; at least two amino acids must be present, the rest may be present or absent
  misc_feature (82)..(96): Xaa can be any naturally occurring amino acid; at least two amino acids must be present, the rest may be present or absent
EVVAATPTSLLISWXXXXXXXXXXXXXXXYRITYGETGGNSPVQEFTVXXXXXXXXXXXXXXXATISGLKPGVDYTITVYAXXXXXXXXXXXXXXXISINYRT

SEQ ID NO: 5 - protein, 86 aa, Artificial Sequence
  Synthetic: ATI-968 core (aka ADX_1760_C01)
EVVAATPTSLLISWIAPFYNVIYYRITYGETGGNSPVQEFTVPGTGYTATISGLKPGVDYTITVYAVTDGASIASYAFPISINYRT

SEQ ID NO: 6 - protein, 9 aa, Artificial Sequence
  Synthetic: ATI-968 BC loop
IAPFYNVIY

SEQ ID NO: 7 - protein, 6 aa, Artificial Sequence
  Synthetic: ATI-968 DE loop
PGTGYT

SEQ ID NO: 8 - protein, 13 aa, Artificial Sequence
  Synthetic: ATI-968 FG loop
VTDGASIASYAFP

SEQ ID NO: 9 - protein, 95 aa, Artificial Sequence
  Synthetic: ATI-968 w/ N leader
GVSDVPRDLEVVAATPTSLLISWIAPFYNVIYYRITYGETGGNSPVQEFTVPGTGYTATISGLKPGVDYTITVYAVTDGASIASYAFPISINYRT

SEQ ID NO: 10 - protein, 101 aa, Artificial Sequence
  Synthetic: ATI-968 w/ N leader + his tag
GVSDVPRDLEVVAATPTSLLISWIAPFYNVIYYRITYGETGGNSPVQEFTVPGTGYTATISGLKPGVDYTITVYAVTDGASIASYAFPISINYRTHHHHHH

SEQ ID NO: 11 - protein, 102 aa, Artificial Sequence
  Synthetic: ATI-968 w/ N leader and C tail
GVSDVPRDLEVVAATPTSLLISWIAPFYNVIYYRITYGETGGNSPVQEFTVPGTGYTATISGLKPGVDYTITVYAVTDGASIASYAFPISINYRTEIDKPSQ

SEQ ID NO: 12 - protein, 108 aa, Artificial Sequence
  Synthetic: ATI-968 w/ N leader and C tail + his tag
GVSDVPRDLEVVAATPTSLLISWIAPFYNVIYYRITYGETGGNSPVQEFTVPGTGYTATISGLKPGVDYTITVYAVTDGASIASYAFPISINYRTEIDKPSQHHHHHH

SEQ ID NO: 13 - protein, 97 aa, Artificial Sequence
  Synthetic: ATI-968 w/ N leader and modified C-terminus including PC
GVSDVPRDLEVVAATPTSLLISWIAPFYNVIYYRITYGETGGNSPVQEFTVPGTGYTATISGLKPGVDYTITVYAVTDGASIASYAFPISINYRTPC

SEQ ID NO: 14 - protein, 103 aa, Artificial Sequence
  Synthetic: ATI-968 w/ N leader and modified C-terminus including PC + his tag
GVSDVPRDLEVVAATPTSLLISWIAPFYNVIYYRITYGETGGNSPVQEFTVPGTGYTATISGLKPGVDYTITVYAVTDGASIASYAFPISINYRTPCHHHHHH

SEQ ID NO: 15 - protein, 109 aa, Artificial Sequence
  Synthetic: ATI-968  full length
MGVSDVPRDLEVVAATPTSLLISWIAPFYNVIYYRITYGETGGNSPVQEFTVPGTGYTATISGLKPGVDYTITVYAVTDGASIASYAFPISINYRTEIDKPSQHHHHHH

SEQ ID NO: 16 - DNA, 258 bp, Artificial Sequence
  Synthetic: ATI-968  core (nucleotide sequence)
gaagtggttgctgccacccccaccagcctgctgatcagctggatcgctccgttctacaatgtcatctattaccgcatcacttacggcgaaacaggaggcaatagccctgtccaggagttcactgtgcctggtactggttatacagctacaatcagcggccttaaacctggcgttgattataccatcactgtgtatgctgtcactgatggagcatccattgcttcatacgcgtttccaatttccattaattaccgcaca

SEQ ID NO: 17 - DNA, 288 bp, Artificial Sequence
  Synthetic: ATI-968 w/ N leader (nucleotide sequence with N-terminal methionine)
atgggagtttctgatgtgccgcgcgacctggaagtggttgctgccacccccaccagcctgctgatcagctggatcgctccgttctacaatgtcatctattaccgcatcacttacggcgaaacaggaggcaatagccctgtccaggagttcactgtgcctggtactggttatacagctacaatcagcggccttaaacctggcgttgattataccatcactgtgtatgctgtcactgatggagcatccattgcttcatacgcgtttccaatttccattaattaccgcaca

SEQ ID NO: 18 - DNA, 294 bp, Artificial Sequence
  Synthetic: ATI-968 w/ N leader and modified C-terminus including PC (nucleotide sequence with N-terminal methionine)
atgggagtttctgatgtgccgcgcgacctggaagtggttgctgccacccccaccagcctgctgatcagctggatcgctccgttctacaatgtcatctattaccgcatcacttacggcgaaacaggaggcaatagccctgtccaggagttcactgtgcctggtactggttatacagctacaatcagcggccttaaacctggcgttgattataccatcactgtgtatgctgtcactgatggagcatccattgcttcatacgcgtttccaatttccattaattaccgcacaccgtgc

SEQ ID NO: 19 - DNA, 330 bp, Artificial Sequence
  Synthetic: ATI-968 w/ N leader and C tail + his tag (nucleotide sequence with N-terminal methionine)
atgggagtttctgatgtgccgcgcgacctggaagtggttgctgccacccccaccagcctgctgatcagctggatcgctccgttctacaatgtcatctattaccgcatcacttacggcgaaacaggaggcaatagccctgtccaggagttcactgtgcctggtactggttatacagctacaatcagcggccttaaacctggcgttgattataccatcactgtgtatgctgtcactgatggagcatccattgcttcatacgcgtttccaatttccattaattaccgcacagaaattgacaaaccatcccagcaccatcaccaccaccactga

SEQ ID NO: 20 - protein, 86 aa, Artificial Sequence
  Synthetic: ATI-964 core (parent of ADX_5322_A02)
EVVAATPTSLLISWSYDGSIERYYRITYGETGGNSPVQEFTVPPDQKTATISGLKPGVDYTITVYAVRLEEAHYYRESPISINYRT

SEQ ID NO: 21 - protein, 9 aa, Artificial Sequence
  Synthetic: ATI-964 BC loop
SYDGSIERY

SEQ ID NO: 22 - protein, 6 aa, Artificial Sequence
  Synthetic: ATI-964 DE loop
PPDQKT

SEQ ID NO: 23 - protein, 13 aa, Artificial Sequence
  Synthetic: ATI-964 FG loop
VRLEEAHYYRESP

SEQ ID NO: 24 - protein, 95 aa, Artificial Sequence
  Synthetic: ATI-964 w/ N leader
GVSDVPRDLEVVAATPTSLLISWSYDGSIERYYRITYGETGGNSPVQEFTVPPDQKTATISGLKPGVDYTITVYAVRLEEAHYYRESPISINYRT

SEQ ID NO: 25 - protein, 101 aa, Artificial Sequence
  Synthetic: ATI-964 w/ N leader + his tag
GVSDVPRDLEVVAATPTSLLISWSYDGSIERYYRITYGETGGNSPVQEFTVPPDQKTATISGLKPGVDYTITVYAVRLEEAHYYRESPISINYRTHHHHHH

SEQ ID NO: 26 - protein, 102 aa, Artificial Sequence
  Synthetic: ATI-964 w/ N leader and C tail
GVSDVPRDLEVVAATPTSLLISWSYDGSIERYYRITYGETGGNSPVQEFTVPPDQKTATISGLKPGVDYTITVYAVRLEEAHYYRESPISINYRTEIDKPSQ

SEQ ID NO: 27 - protein, 108 aa, Artificial Sequence
  Synthetic: ATI-964 w/ N leader and C tail + his tag
GVSDVPRDLEVVAATPTSLLISWSYDGSIERYYRITYGETGGNSPVQEFTVPPDQKTATISGLKPGVDYTITVYAVRLEEAHYYRESPISINYRTEIDKPSQHHHHHH

SEQ ID NO: 28 - protein, 97 aa, Artificial Sequence
  Synthetic: ATI-964 w/ N leader and modified C-terminus including PC
GVSDVPRDLEVVAATPTSLLISWSYDGSIERYYRITYGETGGNSPVQEFTVPPDQKTATISGLKPGVDYTITVYAVRLEEAHYYRESPISINYRTPC

SEQ ID NO: 29 - protein, 103 aa, Artificial Sequence
  Synthetic: ATI-964 w/ N leader and modified C-terminus including PC + his tag
GVSDVPRDLEVVAATPTSLLISWSYDGSIERYYRITYGETGGNSPVQEFTVPPDQKTATISGLKPGVDYTITVYAVRLEEAHYYRESPISINYRTPCHHHHHH

SEQ ID NO: 30 - protein, 109 aa, Artificial Sequence
  Synthetic: ATI-964  full length
MGVSDVPRDLEVVAATPTSLLISWSYDGSIERYYRITYGETGGNSPVQEFTVPPDQKTATISGLKPGVDYTITVYAVRLEEAHYYRESPISINYRTEIDKPSQHHHHHH

SEQ ID NO: 31 - DNA, 258 bp, Artificial Sequence
  Synthetic: ATI-964  core (nucleotide sequence)
gaagtggttgctgccacccccaccagcctgctgatcagctggtcttacgacggttcgattgaacgttattaccgcatcacttacggcgaaacaggaggcaatagccctgtccaggagttcactgtgcctccggatcagaagacagctaccatcagcggccttaaacctggcgttgattataccatcactgtgtatgctgtcaggctggaagaagctcattactatcgagagtctccaatttccattaattaccgcaca

SEQ ID NO: 32 - DNA, 288 bp, Artificial Sequence
  Synthetic: ATI-964 w/ N leader (nucleotide sequence with N-terminal methionine)
atgggagtttctgatgtgccgcgcgacctggaagtggttgctgccacccccaccagcctgctgatcagctggtcttacgacggttcgattgaacgttattaccgcatcacttacggcgaaacaggaggcaatagccctgtccaggagttcactgtgcctccggatcagaagacagctaccatcagcggccttaaacctggcgttgattataccatcactgtgtatgctgtcaggctggaagaagctcattactatcgagagtctccaatttccattaattaccgcaca

SEQ ID NO: 33 - DNA, 294 bp, Artificial Sequence
  Synthetic: ATI-964 w/ N leader and modified C-terminus including PC (nucleotide sequence with N-terminal methionine)
atgggagtttctgatgtgccgcgcgacctggaagtggttgctgccacccccaccagcctgctgatcagctggtcttacgacggttcgattgaacgttattaccgcatcacttacggcgaaacaggaggcaatagccctgtccaggagttcactgtgcctccggatcagaagacagctaccatcagcggccttaaacctggcgttgattataccatcactgtgtatgctgtcaggctggaagaagctcattactatcgagagtctccaatttccattaattaccgcacaccgtgc

SEQ ID NO: 34 - DNA, 330 bp, Artificial Sequence
  Synthetic: ATI-964 w/ N leader and C tail + his tag (nucleotide sequence with N-terminal methionine)
atgggagtttctgatgtgccgcgcgacctggaagtggttgctgccacccccaccagcctgctgatcagctggtcttacgacggttcgattgaacgttattaccgcatcacttacggcgaaacaggaggcaatagccctgtccaggagttcactgtgcctccggatcagaagacagctaccatcagcggccttaaacctggcgttgattataccatcactgtgtatgctgtcaggctggaagaagctcattactatcgagagtctccaatttccattaattaccgcacagaaattgacaaaccatcccagcaccatcaccaccaccactga

SEQ ID NO: 35 - protein, 86 aa, Artificial Sequence
  Synthetic: ATI-965 core
EVVAATPTSLLISWTAYDSVDKYYRITYGETGGNSPVQEFTVGPRHHTATISGLKPGVDYTITVYAVYHTEPGYHAHMPISINYRT

SEQ ID NO: 36 - protein, 9 aa, Artificial Sequence
  Synthetic: ATI-965 BC loop
TAYDSVDKY

SEQ ID NO: 37 - protein, 6 aa, Artificial Sequence
  Synthetic: ATI-965 DE loop
GPRHHT

SEQ ID NO: 38 - protein, 13 aa, Artificial Sequence
  Synthetic: ATI-965 FG loop
VYHTEPGYHAHMP

SEQ ID NO: 39 - protein, 95 aa, Artificial Sequence
  Synthetic: ATI-965 w/ N leader
GVSDVPRDLEVVAATPTSLLISWTAYDSVDKYYRITYGETGGNSPVQEFTVGPRHHTATISGLKPGVDYTITVYAVYHTEPGYHAHMPISINYRT

SEQ ID NO: 40 - protein, 101 aa, Artificial Sequence
  Synthetic: ATI-965 w/ N leader + his tag
GVSDVPRDLEVVAATPTSLLISWTAYDSVDKYYRITYGETGGNSPVQEFTVGPRHHTATISGLKPGVDYTITVYAVYHTEPGYHAHMPISINYRTHHHHHH

SEQ ID NO: 41 - protein, 102 aa, Artificial Sequence
  Synthetic: ATI-965 w/ N leader and C tail
GVSDVPRDLEVVAATPTSLLISWTAYDSVDKYYRITYGETGGNSPVQEFTVGPRHHTATISGLKPGVDYTITVYAVYHTEPGYHAHMPISINYRTEIDKPSQ

SEQ ID NO: 42 - protein, 108 aa, Artificial Sequence
  Synthetic: ATI-965 w/ N leader and C tail + his tag
GVSDVPRDLEVVAATPTSLLISWTAYDSVDKYYRITYGETGGNSPVQEFTVGPRHHTATISGLKPGVDYTITVYAVYHTEPGYHAHMPISINYRTEIDKPSQHHHHHH

SEQ ID NO: 43 - protein, 97 aa, Artificial Sequence
  Synthetic: ATI-965 w/ N leader and modified C-terminus including PC
GVSDVPRDLEVVAATPTSLLISWTAYDSVDKYYRITYGETGGNSPVQEFTVGPRHHTATISGLKPGVDYTITVYAVYHTEPGYHAHMPISINYRTPC

SEQ ID NO: 44 - protein, 103 aa, Artificial Sequence
  Synthetic: ATI-965 w/ N leader and modified C-terminus including PC + his tag
GVSDVPRDLEVVAATPTSLLISWTAYDSVDKYYRITYGETGGNSPVQEFTVGPRHHTATISGLKPGVDYTITVYAVYHTEPGYHAHMPISINYRTPCHHHHHH

SEQ ID NO: 45 - protein, 109 aa, Artificial Sequence
  Synthetic: ATI-965  full length
MGVSDVPRDLEVVAATPTSLLISWTAYDSVDKYYRITYGETGGNSPVQEFTVGPRHHTATISGLKPGVDYTITVYAVYHTEPGYHAHMPISINYRTEIDKPSQHHHHHH

SEQ ID NO: 46 - DNA, 258 bp, Artificial Sequence
  Synthetic: ATI-965  core (nucleotide sequence)
gaagtggttgctgccacccccaccagcctgctgatcagctggactgcatacgactctgttgacaaatattaccgcatcacttacggcgaaacaggaggcaatagccctgtccaggagttcactgtgggccctagacatcacacagctaccatcagcggccttaaacctggcgttgattataccatcactgtgtatgctgtctatcacactgaaccgggctatcatgctcatatgccaatttccattaattaccgcaca

SEQ ID NO: 47 - DNA, 288 bp, Artificial Sequence
  Synthetic: ATI-965 w/ N leader (nucleotide sequence with N-terminal methionine)
atgggagtttctgatgtgccgcgcgacctggaagtggttgctgccacccccaccagcctgctgatcagctggactgcatacgactctgttgacaaatattaccgcatcacttacggcgaaacaggaggcaatagccctgtccaggagttcactgtgggccctagacatcacacagctaccatcagcggccttaaacctggcgttgattataccatcactgtgtatgctgtctatcacactgaaccgggctatcatgctcatatgccaatttccattaattaccgcaca

SEQ ID NO: 48 - DNA, 294 bp, Artificial Sequence
  Synthetic: ATI-965 w/ N leader and modified C-terminus including PC (nucleotide sequence with N-terminal methionine)
atgggagtttctgatgtgccgcgcgacctggaagtggttgctgccacccccaccagcctgctgatcagctggactgcatacgactctgttgacaaatattaccgcatcacttacggcgaaacaggaggcaatagccctgtccaggagttcactgtgggccctagacatcacacagctaccatcagcggccttaaacctggcgttgattataccatcactgtgtatgctgtctatcacactgaaccgggctatcatgctcatatgccaatttccattaattaccgcacaccgtgc

SEQ ID NO: 49 - DNA, 330 bp, Artificial Sequence
  Synthetic: ATI-965 w/ N leader and C tail + his tag (nucleotide sequence with N-terminal methionine)
atgggagtttctgatgtgccgcgcgacctggaagtggttgctgccacccccaccagcctgctgatcagctggactgcatacgactctgttgacaaatattaccgcatcacttacggcgaaacaggaggcaatagccctgtccaggagttcactgtgggccctagacatcacacagctaccatcagcggccttaaacctggcgttgattataccatcactgtgtatgctgtctatcacactgaaccgggctatcatgctcatatgccaatttccattaattaccgcacagaaattgacaaaccatcccagcaccatcaccaccaccactga

SEQ ID NO: 50 - protein, 82 aa, Artificial Sequence
  Synthetic: ATI-966 core
EVVAATPTSLLISWHRFSSIMAYYRITYGETGGNSPVQEFTVAGSVNTATISGLKPGVDYTITVYAVTIHNVSFPISINYRT

SEQ ID NO: 51 - protein, 9 aa, Artificial Sequence
  Synthetic: ATI-966 BC loop
HRFSSIMAY

SEQ ID NO: 52 - protein, 6 aa, Artificial Sequence
  Synthetic: ATI-966 DE loop
AGSVNT

SEQ ID NO: 53 - protein, 9 aa, Artificial Sequence
  Synthetic: ATI-966 FG loop
VTIHNVSFP

SEQ ID NO: 54 - protein, 91 aa, Artificial Sequence
  Synthetic: ATI-966 w/ N leader
GVSDVPRDLEVVAATPTSLLISWHRFSSIMAYYRITYGETGGNSPVQEFTVAGSVNTATISGLKPGVDYTITVYAVTIHNVSFPISINYRT

SEQ ID NO: 55 - protein, 97 aa, Artificial Sequence
  Synthetic: ATI-966 w/ N leader + his tag
GVSDVPRDLEVVAATPTSLLISWHRFSSIMAYYRITYGETGGNSPVQEFTVAGSVNTATISGLKPGVDYTITVYAVTIHNVSFPISINYRTHHHHHH

SEQ ID NO: 56 - protein, 98 aa, Artificial Sequence
  Synthetic: ATI-966 w/ N leader and C tail
GVSDVPRDLEVVAATPTSLLISWHRFSSIMAYYRITYGETGGNSPVQEFTVAGSVNTATISGLKPGVDYTITVYAVTIHNVSFPISINYRTEIDKPSQ

SEQ ID NO: 57 - protein, 104 aa, Artificial Sequence
  Synthetic: ATI-966 w/ N leader and C tail + his tag
GVSDVPRDLEVVAATPTSLLISWHRFSSIMAYYRITYGETGGNSPVQEFTVAGSVNTATISGLKPGVDYTITVYAVTIHNVSFPISINYRTEIDKPSQHHHHHH

SEQ ID NO: 58 - protein, 93 aa, Artificial Sequence
  Synthetic: ATI-966 w/ N leader and modified C-terminus including PC
GVSDVPRDLEVVAATPTSLLISWHRFSSIMAYYRITYGETGGNSPVQEFTVAGSVNTATISGLKPGVDYTITVYAVTIHNVSFPISINYRTPC

SEQ ID NO: 59 - protein, 99 aa, Artificial Sequence
  Synthetic: ATI-966 w/ N leader and modified C-terminus including PC + his tag
GVSDVPRDLEVVAATPTSLLISWHRFSSIMAYYRITYGETGGNSPVQEFTVAGSVNTATISGLKPGVDYTITVYAVTIHNVSFPISINYRTPCHHHHHH

SEQ ID NO: 60 - protein, 105 aa, Artificial Sequence
  Synthetic: ATI-966  full length
MGVSDVPRDLEVVAATPTSLLISWHRFSSIMAYYRITYGETGGNSPVQEFTVAGSVNTATISGLKPGVDYTITVYAVTIHNVSFPISINYRTEIDKPSQHHHHHH

SEQ ID NO: 61 - DNA, 246 bp, Artificial Sequence
  Synthetic: ATI-966  core (nucleotide sequence)
gaagtggttgctgccacccccaccagcctgctgatcagctggcataggttctcttctatcatggcgtattaccgcatcacttacggcgaaacaggaggcaatagccctgtccaggagttcactgtggctggctctgttaacacagctaccatcagcggccttaaacctggcgttgattataccatcactgtgtatgctgtcacgatccataacgtttctttcccaatttccattaattaccgcaca

SEQ ID NO: 62 - DNA, 276 bp, Artificial Sequence
  Synthetic: ATI-966w/ N leader (nucleotide sequence with N-terminal methionine)
atgggagtttctgatgtgccgcgcgacctggaagtggttgctgccacccccaccagcctgctgatcagctggcataggttctcttctatcatggcgtattaccgcatcacttacggcgaaacaggaggcaatagccctgtccaggagttcactgtggctggctctgttaacacagctaccatcagcggccttaaacctggcgttgattataccatcactgtgtatgctgtcacgatccataacgtttctttcccaatttccattaattaccgcaca

SEQ ID NO: 63 - DNA, 282 bp, Artificial Sequence
  Synthetic: ATI-966 w/ N leader and modified C-terminus including PC (nucleotide sequence with N-terminal methionine)
atgggagtttctgatgtgccgcgcgacctggaagtggttgctgccacccccaccagcctgctgatcagctggcataggttctcttctatcatggcgtattaccgcatcacttacggcgaaacaggaggcaatagccctgtccaggagttcactgtggctggctctgttaacacagctaccatcagcggccttaaacctggcgttgattataccatcactgtgtatgctgtcacgatccataacgtttctttcccaatttccattaattaccgcacaccgtgc

SEQ ID NO: 64 - DNA, 318 bp, Artificial Sequence
  Synthetic: ATI-966 w/ N leader and C tail + his tag (nucleotide sequence with N-terminal methionine)
atgggagtttctgatgtgccgcgcgacctggaagtggttgctgccacccccaccagcctgctgatcagctggcataggttctcttctatcatggcgtattaccgcatcacttacggcgaaacaggaggcaatagccctgtccaggagttcactgtggctggctctgttaacacagctaccatcagcggccttaaacctggcgttgattataccatcactgtgtatgctgtcacgatccataacgtttctttcccaatttccattaattaccgcacagaaattgacaaaccatcccagcaccatcaccaccaccactga

SEQ ID NO: 65 - protein, 84 aa, Artificial Sequence
  Synthetic: ATI-967 core (parent of ADX_5417_E01)
EVVAATPTSLLISWQGQLSPSFYYRITYGETGGNSPVQEFTVPVASGTATISGLKPGVDYTITVYAVTSHGIYFYAPISINYRT

SEQ ID NO: 66 - protein, 9 aa, Artificial Sequence
  Synthetic: ATI-967 BC loop
QGQLSPSFY

SEQ ID NO: 67 - protein, 6 aa, Artificial Sequence
  Synthetic: ATI-967 DE loop
PVASGT

SEQ ID NO: 68 - protein, 11 aa, Artificial Sequence
  Synthetic: ATI-967 FG loop
VTSHGIYFYAP

SEQ ID NO: 69 - protein, 93 aa, Artificial Sequence
  Synthetic: ATI-967 w/ N leader
GVSDVPRDLEVVAATPTSLLISWQGQLSPSFYYRITYGETGGNSPVQEFTVPVASGTATISGLKPGVDYTITVYAVTSHGIYFYAPISINYRT

SEQ ID NO: 70 - protein, 99 aa, Artificial Sequence
  Synthetic: ATI-967 w/ N leader + his tag
GVSDVPRDLEVVAATPTSLLISWQGQLSPSFYYRITYGETGGNSPVQEFTVPVASGTATISGLKPGVDYTITVYAVTSHGIYFYAPISINYRTHHHHHH

SEQ ID NO: 71 - protein, 100 aa, Artificial Sequence
  Synthetic: ATI-967 w/ N leader and C tail
GVSDVPRDLEVVAATPTSLLISWQGQLSPSFYYRITYGETGGNSPVQEFTVPVASGTATISGLKPGVDYTITVYAVTSHGIYFYAPISINYRTEIDKPSQ

SEQ ID NO: 72 - protein, 106 aa, Artificial Sequence
  Synthetic: ATI-967 w/ N leader and C tail + his tag
GVSDVPRDLEVVAATPTSLLISWQGQLSPSFYYRITYGETGGNSPVQEFTVPVASGTATISGLKPGVDYTITVYAVTSHGIYFYAPISINYRTEIDKPSQHHHHHH

SEQ ID NO: 73 - protein, 95 aa, Artificial Sequence
  Synthetic: ATI-967 w/ N leader and modified C-terminus including PC
GVSDVPRDLEVVAATPTSLLISWQGQLSPSFYYRITYGETGGNSPVQEFTVPVASGTATISGLKPGVDYTITVYAVTSHGIYFYAPISINYRTPC

SEQ ID NO: 74 - protein, 101 aa, Artificial Sequence
  Synthetic: ATI-967 w/ N leader and modified C-terminus including PC + his tag
GVSDVPRDLEVVAATPTSLLISWQGQLSPSFYYRITYGETGGNSPVQEFTVPVASGTATISGLKPGVDYTITVYAVTSHGIYFYAPISINYRTPCHHHHHH

SEQ ID NO: 75 - protein, 107 aa, Artificial Sequence
  Synthetic: ATI-967  full length
MGVSDVPRDLEVVAATPTSLLISWQGQLSPSFYYRITYGETGGNSPVQEFTVPVASGTATISGLKPGVDYTITVYAVTSHGIYFYAPISINYRTEIDKPSQHHHHHH

SEQ ID NO: 76 - DNA, 252 bp, Artificial Sequence
  Synthetic: ATI-967  core (nucleotide sequence)
gaagtggttgctgccacccccaccagcctgctgatcagctggcagggacagctgtctccgtctttctattaccgaatcacttacggcgaaacaggaggcaatagccctgtccaggagttcactgtgcctgttgctagtgggacagctaccatcagcggccttaaacctggcgttgattataccatcactgtgtatgctgtcacttctcatggcatatacttctacgctccaatttccattaattaccgcaca

SEQ ID NO: 77 - DNA, 282 bp, Artificial Sequence
  Synthetic: ATI-967 w/ N leader (nucleotide sequence with N-terminal methionine)
atgggagtttctgatgtgccgcgcgacctggaagtggttgctgccacccccaccagcctgctgatcagctggcagggacagctgtctccgtctttctattaccgaatcacttacggcgaaacaggaggcaatagccctgtccaggagttcactgtgcctgttgctagtgggacagctaccatcagcggccttaaacctggcgttgattataccatcactgtgtatgctgtcacttctcatggcatatacttctacgctccaatttccattaattaccgcaca

SEQ ID NO: 78 - DNA, 288 bp, Artificial Sequence
  Synthetic: ATI-967 w/ N leader and modified C-terminus including PC (nucleotide sequence with N-terminal methionine)
atgggagtttctgatgtgccgcgcgacctggaagtggttgctgccacccccaccagcctgctgatcagctggcagggacagctgtctccgtctttctattaccgaatcacttacggcgaaacaggaggcaatagccctgtccaggagttcactgtgcctgttgctagtgggacagctaccatcagcggccttaaacctggcgttgattataccatcactgtgtatgctgtcacttctcatggcatatacttctacgctccaatttccattaattaccgcacaccgtgc

SEQ ID NO: 79 - DNA, 325 bp, Artificial Sequence
  Synthetic: ATI-967 w/ N leader and C tail + his tag (nucleotide sequence with N-terminal methionine)
atgggagtttctgatgtgccgcgcgacctggaagtggttgctgccacccccaccagcctgctgatcagctggcagggacagctgtctccgtctttctattaccgaatcacttacggcgaaacaggaggcaatagccctgtccaggagttcactgtgcctgttgctagtgggacagctaccatcagcggccttaaacctggcgttgattataccatcactgtgtatgctgtcacttctcatggcatatacttctacgctccaatttccattaattaccgcacagaaattgacaaaccatcccagcaccatcaccaccaccactgat

SEQ ID NO: 80 - protein, 86 aa, Artificial Sequence
  Synthetic: ADX_5322_A02 core
EVVAATPTSLLISWSYDGPIDRYYRITYGETGGNSPVQEFTVPPDQKTATISGLKPGVDYTITVYAVRLEEAHYNREFPISINYRT

SEQ ID NO: 81 - protein, 9 aa, Artificial Sequence
  Synthetic: ADX_5322_A02  BC loop
SYDGPIDRY

SEQ ID NO: 82 - protein, 6 aa, Artificial Sequence
  Synthetic: ADX_5322_A02  DE loop
PPDQKT

SEQ ID NO: 83 - protein, 13 aa, Artificial Sequence
  Synthetic: ADX_5322_A02  FG loop
VRLEEAHYNREFP

SEQ ID NO: 84 - protein, 95 aa, Artificial Sequence
  Synthetic: ADX_5322_A02  w/ N leader
GVSDVPRDLEVVAATPTSLLISWSYDGPIDRYYRITYGETGGNSPVQEFTVPPDQKTATISGLKPGVDYTITVYAVRLEEAHYNREFPISINYRT

SEQ ID NO: 85 - protein, 101 aa, Artificial Sequence
  Synthetic: ADX_5322_A02  w/ N leader + his tag
GVSDVPRDLEVVAATPTSLLISWSYDGPIDRYYRITYGETGGNSPVQEFTVPPDQKTATISGLKPGVDYTITVYAVRLEEAHYNREFPISINYRTHHHHHH

SEQ ID NO: 86 - protein, 102 aa, Artificial Sequence
  Synthetic: ADX_5322_A02  w/ N leader and C tail
GVSDVPRDLEVVAATPTSLLISWSYDGPIDRYYRITYGETGGNSPVQEFTVPPDQKTATISGLKPGVDYTITVYAVRLEEAHYNREFPISINYRTEIDKPSQ

SEQ ID NO: 87 - protein, 108 aa, Artificial Sequence
  Synthetic: ADX_5322_A02  w/ N leader and C tail + his tag
GVSDVPRDLEVVAATPTSLLISWSYDGPIDRYYRITYGETGGNSPVQEFTVPPDQKTATISGLKPGVDYTITVYAVRLEEAHYNREFPISINYRTEIDKPSQHHHHHH

SEQ ID NO: 88 - protein, 97 aa, Artificial Sequence
  Synthetic: ADX_5322_A02  w/ N leader and modified C-terminus including PC
GVSDVPRDLEVVAATPTSLLISWSYDGPIDRYYRITYGETGGNSPVQEFTVPPDQKTATISGLKPGVDYTITVYAVRLEEAHYNREFPISINYRTPC

SEQ ID NO: 89 - protein, 103 aa, Artificial Sequence
  Synthetic: ADX_5322_A02  w/ N leader and modified C-terminus including PC + his tag
GVSDVPRDLEVVAATPTSLLISWSYDGPIDRYYRITYGETGGNSPVQEFTVPPDQKTATISGLKPGVDYTITVYAVRLEEAHYNREFPISINYRTPCHHHHHH

SEQ ID NO: 90 - protein, 97 aa, Artificial Sequence; identical to SEQ ID NO: 88
  Synthetic: ADX_5322_A02-Mal-DBCO-FFPF18

SEQ ID NO: 91 - protein, 104 aa, Artificial Sequence
  Synthetic: ADX_5322_A02 full length
MGVSDVPRDLEVVAATPTSLLISWSYDGPIDRYYRITYGETGGNSPVQEFTVPPDQKTATISGLKPGVDYTITVYAVRLEEAHYNREFPISINYRTPCHHHHHH

SEQ ID NO: 92 - DNA, 258 bp, Artificial Sequence
  Synthetic: ADX_5322_A02  core (nucleotide sequence)
gaagtggttgctgccacccccaccagcctgctgatcagctggtcttacgatggcccaattgaccggtattaccgcatcacttacggcgaaacaggaggcaatagccctgtccaggagttcactgtgcctccggatcagaagacagctaccatcagcggccttaaacctggcgttgattataccatcactgtgtatgctgtccggctggaagaagctcattacaatcgagagtttccaatttccattaattaccgcaca

SEQ ID NO: 93 - DNA, 288 bp, Artificial Sequence
  Synthetic: ADX_5322_A02 w/ N leader (nucleotide sequence with N-terminal methionine)
atgggagtttctgatgtgccgcgcgacctggaagtggttgctgccacccccaccagcctgctgatcagctggtcttacgatggcccaattgaccggtattaccgcatcacttacggcgaaacaggaggcaatagccctgtccaggagttcactgtgcctccggatcagaagacagctaccatcagcggccttaaacctggcgttgattataccatcactgtgtatgctgtccggctggaagaagctcattacaatcgagagtttccaatttccattaattaccgcaca

SEQ ID NO: 94 - DNA, 294 bp, Artificial Sequence
  Synthetic: ADX_5322_A02 w/ N leader and modified C-terminus including PC (nucleotide sequence with N-terminal methionine)
atgggagtttctgatgtgccgcgcgacctggaagtggttgctgccacccccaccagcctgctgatcagctggtcttacgatggcccaattgaccggtattaccgcatcacttacggcgaaacaggaggcaatagccctgtccaggagttcactgtgcctccggatcagaagacagctaccatcagcggccttaaacctggcgttgattataccatcactgtgtatgctgtccggctggaagaagctcattacaatcgagagtttccaatttccattaattaccgcacaccgtgc

SEQ ID NO: 95 - DNA, 315 bp, Artificial Sequence
  Synthetic: ADX_5322_A02 w/ N leader and C tail + his tag (nucleotide sequence with N-terminal methionine)
atgggagtttctgatgtgccgcgcgacctggaagtggttgctgccacccccaccagcctgctgatcagctggtcttacgatggcccaattgaccggtattaccgcatcacttacggcgaaacaggaggcaatagccctgtccaggagttcactgtgcctccggatcagaagacagctaccatcagcggccttaaacctggcgttgattataccatcactgtgtatgctgtccggctggaagaagctcattacaatcgagagtttccaatttccattaattaccgcacaccgtgccaccatcaccaccaccactga

SEQ ID NO: 96 - protein, 84 aa, Artificial Sequence
  Synthetic: ADX_5417_E01 core
EVVAATPTSLLISWRAQLSPSFYYRITYGETGGNSPVQEFTVPNDVMTATISGLKPGVDYTITVYAVTTHGVYFYSPISINYRT

SEQ ID NO: 97 - protein, 9 aa, Artificial Sequence
  Synthetic: ADX_5417_E01 BC loop
RAQLSPSFY

SEQ ID NO: 98 - protein, 6 aa, Artificial Sequence
  Synthetic: ADX_5417_E01 DE loop
PNDVMT

SEQ ID NO: 99 - protein, 11 aa, Artificial Sequence
  Synthetic: ADX_5417_E01 FG loop
VTTHGVYFYSP

SEQ ID NO: 100 - protein, 93 aa, Artificial Sequence
  Synthetic: ADX_5417_E01 w/ N leader
GVSDVPRDLEVVAATPTSLLISWRAQLSPSFYYRITYGETGGNSPVQEFTVPNDVMTATISGLKPGVDYTITVYAVTTHGVYFYSPISINYRT

SEQ ID NO: 101 - protein, 99 aa, Artificial Sequence
  Synthetic: ADX_5417_E01 w/ N leader + his tag
GVSDVPRDLEVVAATPTSLLISWRAQLSPSFYYRITYGETGGNSPVQEFTVPNDVMTATISGLKPGVDYTITVYAVTTHGVYFYSPISINYRTHHHHHH

SEQ ID NO: 102 - protein, 100 aa, Artificial Sequence
  Synthetic: ADX_5417_E01 w/ N leader and C tail
GVSDVPRDLEVVAATPTSLLISWRAQLSPSFYYRITYGETGGNSPVQEFTVPNDVMTATISGLKPGVDYTITVYAVTTHGVYFYSPISINYRTEIDKPSQ

SEQ ID NO: 103 - protein, 106 aa, Artificial Sequence
  Synthetic: ADX_5417_E01 w/ N leader and C tail + his tag
GVSDVPRDLEVVAATPTSLLISWRAQLSPSFYYRITYGETGGNSPVQEFTVPNDVMTATISGLKPGVDYTITVYAVTTHGVYFYSPISINYRTEIDKPSQHHHHHH

SEQ ID NO: 104 - protein, 95 aa, Artificial Sequence
  Synthetic: ADX_5417_E01 w/ N leader and modified C-terminus including PC
GVSDVPRDLEVVAATPTSLLISWRAQLSPSFYYRITYGETGGNSPVQEFTVPNDVMTATISGLKPGVDYTITVYAVTTHGVYFYSPISINYRTPC

SEQ ID NO: 105 - protein, 101 aa, Artificial Sequence
  Synthetic: ADX_5417_E01 w/ N leader and modified C-terminus including PC + his tag
GVSDVPRDLEVVAATPTSLLISWRAQLSPSFYYRITYGETGGNSPVQEFTVPNDVMTATISGLKPGVDYTITVYAVTTHGVYFYSPISINYRTPCHHHHHH

SEQ ID NO: 106 - protein, 97 aa, Artificial Sequence; identical to SEQ ID NO: 88
  Synthetic: ADX-5417_E01 Mal-DBCO-FFPF18

SEQ ID NO: 107 - protein, 102 aa, Artificial Sequence
  Synthetic: ADX-5417_E01 full length
MGVSDVPRDLEVVAATPTSLLISWRAQLSPSFYYRITYGETGGNSPVQEFTVPNDVMTATISGLKPGVDYTITVYAVTTHGVYFYSPISINYRTPCHHHHHH

SEQ ID NO: 108 - DNA, 252 bp, Artificial Sequence
  Synthetic: ADX-5417_E01  core (nucleotide sequence)
gaagtggttgctgccacccccaccagcctgctgatcagctggagggctcagctgtctccgtctttctattaccgcatcacttacggcgaaacaggaggcaatagccctgtccaggagttcactgtgcctaatgatgtaatgacagctaccatcagcggccttaaacctggcgttgattataccatcactgtgtatgctgtcactactcatggtgtttatttctactcaccaatttccattaattaccgcaca

SEQ ID NO: 109 - DNA, 282 bp, Artificial Sequence
  Synthetic: ADX_5417_E01 w/ N leader (nucleotide sequence with N-terminal methionine)
atgggagtttctgatgtgccgcgcgacctggaagtggttgctgccacccccaccagcctgctgatcagctggagggctcagctgtctccgtctttctattaccgcatcacttacggcgaaacaggaggcaatagccctgtccaggagttcactgtgcctaatgatgtaatgacagctaccatcagcggccttaaacctggcgttgattataccatcactgtgtatgctgtcactactcatggtgtttatttctactcaccaatttccattaattaccgcaca

SEQ ID NO: 110 - DNA, 288 bp, Artificial Sequence
  Synthetic: ADX_5417_E01 w/ N leader and modified C-terminus including PC (nucleotide sequence with N-terminal methionine)
atgggagtttctgatgtgccgcgcgacctggaagtggttgctgccacccccaccagcctgctgatcagctggagggctcagctgtctccgtctttctattaccgcatcacttacggcgaaacaggaggcaatagccctgtccaggagttcactgtgcctaatgatgtaatgacagctaccatcagcggccttaaacctggcgttgattataccatcactgtgtatgctgtcactactcatggtgtttatttctactcaccaatttccattaattaccgcacaccgtgc

SEQ ID NO: 111 - DNA, 309 bp, Artificial Sequence
  Synthetic: ADX_5417_E01 w/ N leader and C tail + his tag (nucleotide sequence with N-terminal methionine)
atgggagtttctgatgtgccgcgcgacctggaagtggttgctgccacccccaccagcctgctgatcagctggagggctcagctgtctccgtctttctattaccgcatcacttacggcgaaacaggaggcaatagccctgtccaggagttcactgtgcctaatgatgtaatgacagctaccatcagcggccttaaacctggcgttgattataccatcactgtgtatgctgtcactactcatggtgtttatttctactcaccaatttccattaattaccgcacaccgtgccaccatcaccaccaccactga

SEQ ID NO: 112 - protein, 80 aa, Artificial Sequence
  Synthetic: ATI_1420_A10 core
EVVAATPTSLLISWPYPSYYIEYRITYGETGGNSPVQEFTVQSMKATISGLKPGVDYTITVYAIRHPGMLEFGISINYRT

SEQ ID NO: 113 - protein, 8 aa, Artificial Sequence
  Synthetic: ATI_1420_A10 BC loop
PYPSYYIE

SEQ ID NO: 114 - protein, 10 aa, Artificial Sequence
  Synthetic: ATI_1420_A10 DE loop
IRHPGMLEFG

SEQ ID NO: 115 - protein, 13 aa, Artificial Sequence
  Synthetic: ATI_1420_A10 FG loop
VTDGASIASYAFP

SEQ ID NO: 116 - protein, 89 aa, Artificial Sequence
  Synthetic: ATI_1420_A10 w/ N leader
GVSDVPRDLEVVAATPTSLLISWPYPSYYIEYRITYGETGGNSPVQEFTVQSMKATISGLKPGVDYTITVYAIRHPGMLEFGISINYRT

SEQ ID NO: 117 - protein, 95 aa, Artificial Sequence
  Synthetic: ATI_1420_A10 w/ N leader + his tag
GVSDVPRDLEVVAATPTSLLISWPYPSYYIEYRITYGETGGNSPVQEFTVQSMKATISGLKPGVDYTITVYAIRHPGMLEFGISINYRTHHHHHH

SEQ ID NO: 118 - protein, 96 aa, Artificial Sequence
  Synthetic: ATI_1420_A10 w/ N leader and C tail
GVSDVPRDLEVVAATPTSLLISWPYPSYYIEYRITYGETGGNSPVQEFTVQSMKATISGLKPGVDYTITVYAIRHPGMLEFGISINYRTEIDKPSQ

SEQ ID NO: 119 - protein, 102 aa, Artificial Sequence
  Synthetic: ATI_1420_A10w/ N leader and C tail + his tag
GVSDVPRDLEVVAATPTSLLISWPYPSYYIEYRITYGETGGNSPVQEFTVQSMKATISGLKPGVDYTITVYAIRHPGMLEFGISINYRTEIDKPSQHHHHHH

SEQ ID NO: 120 - protein, 91 aa, Artificial Sequence
  Synthetic: ATI_1420_A10w/ N leader and modified C-terminus including PC
GVSDVPRDLEVVAATPTSLLISWPYPSYYIEYRITYGETGGNSPVQEFTVQSMKATISGLKPGVDYTITVYAIRHPGMLEFGISINYRTPC

SEQ ID NO: 121 - protein, 97 aa, Artificial Sequence
  Synthetic: ATI_1420_A10 w/ N leader and modified C-terminus including PC + his tag
GVSDVPRDLEVVAATPTSLLISWPYPSYYIEYRITYGETGGNSPVQEFTVQSMKATISGLKPGVDYTITVYAIRHPGMLEFGISINYRTPCHHHHHH

SEQ ID NO: 122 - protein, 103 aa, Artificial Sequence
  Synthetic: ATI_1420_A10 full length
MGVSDVPRDLEVVAATPTSLLISWPYPSYYIEYRITYGETGGNSPVQEFTVQSMKATISGLKPGVDYTITVYAIRHPGMLEFGISINYRTEIDKPSQHHHHHH

SEQ ID NO: 123 - protein, 76 aa, Artificial Sequence
  Synthetic: ATI_1420_B09 core
EVVAATPTSLLISWHKFSSLMSYRITYGETGGNSPVQEFTVGSVNATISGLKPGVDYTITVYAIHNVGFISINYRT

SEQ ID NO: 124 - protein, 8 aa, Artificial Sequence
  Synthetic: ATI_1420_B09 BC loop
HKFSSLMS

SEQ ID NO: 125 - protein, 4 aa, Artificial Sequence
  Synthetic: ATI_1420_B09 DE loop
GSVN

SEQ ID NO: 126 - protein, 6 aa, Artificial Sequence
  Synthetic: ATI_1420_B09 FG loop
IHNVGF

SEQ ID NO: 127 - protein, 85 aa, Artificial Sequence
  Synthetic: ATI_1420_B09 w/ N leader
GVSDVPRDLEVVAATPTSLLISWHKFSSLMSYRITYGETGGNSPVQEFTVGSVNATISGLKPGVDYTITVYAIHNVGFISINYRT

SEQ ID NO: 128 - protein, 91 aa, Artificial Sequence
  Synthetic: ATI_1420_B09 w/ N leader + his tag
GVSDVPRDLEVVAATPTSLLISWHKFSSLMSYRITYGETGGNSPVQEFTVGSVNATISGLKPGVDYTITVYAIHNVGFISINYRTHHHHHH

SEQ ID NO: 129 - protein, 92 aa, Artificial Sequence
  Synthetic: AATI_1420_B09 w/ N leader and C tail
GVSDVPRDLEVVAATPTSLLISWHKFSSLMSYRITYGETGGNSPVQEFTVGSVNATISGLKPGVDYTITVYAIHNVGFISINYRTEIDKPSQ

SEQ ID NO: 130 - protein, 98 aa, Artificial Sequence
  Synthetic: ATI_1420_B09 w/ N leader and C tail + his tag
GVSDVPRDLEVVAATPTSLLISWHKFSSLMSYRITYGETGGNSPVQEFTVGSVNATISGLKPGVDYTITVYAIHNVGFISINYRTEIDKPSQHHHHHH

SEQ ID NO: 131 - protein, 87 aa, Artificial Sequence
  Synthetic: ATI_1420_B09 w/ N leader and modified C-terminus including PC
GVSDVPRDLEVVAATPTSLLISWHKFSSLMSYRITYGETGGNSPVQEFTVGSVNATISGLKPGVDYTITVYAIHNVGFISINYRTPC

SEQ ID NO: 132 - protein, 93 aa, Artificial Sequence
  Synthetic: ATI_1420_B09 w/ N leader and modified C-terminus including PC + his tag
GVSDVPRDLEVVAATPTSLLISWHKFSSLMSYRITYGETGGNSPVQEFTVGSVNATISGLKPGVDYTITVYAIHNVGFISINYRTPCHHHHHH

SEQ ID NO: 133 - protein, 99 aa, Artificial Sequence
  Synthetic: ATI_1420_B09 full length
MGVSDVPRDLEVVAATPTSLLISWHKFSSLMSYRITYGETGGNSPVQEFTVGSVNATISGLKPGVDYTITVYAIHNVGFISINYRTEIDKPSQHHHHHH

SEQ ID NO: 134 - protein, 79 aa, Artificial Sequence
  Synthetic: ATI_1420_C02 core
EVVAATPTSLLISWRIKSYYAYRITYGETGGNSPVQEFTVRQHVATISGLKPGVDYTITVYARLGDVELVYEISINYRT

SEQ ID NO: 135 - protein, 7 aa, Artificial Sequence
  Synthetic: ATI_1420_C02 BC loop
RIKSYYA

SEQ ID NO: 136 - protein, 4 aa, Artificial Sequence
  Synthetic: ATI_1420_C02 DE loop
RQHV

SEQ ID NO: 137 - protein, 10 aa, Artificial Sequence
  Synthetic: ATI_1420_C02 FG loop
RLGDVELVYE

SEQ ID NO: 138 - protein, 88 aa, Artificial Sequence
  Synthetic: ATI_1420_C02 w/ N leader
GVSDVPRDLEVVAATPTSLLISWRIKSYYAYRITYGETGGNSPVQEFTVRQHVATISGLKPGVDYTITVYARLGDVELVYEISINYRT

SEQ ID NO: 139 - protein, 91 aa, Artificial Sequence; identical to SEQ ID NO: 128
  Synthetic: ATI_1420_C02 w/ N leader + his tag

SEQ ID NO: 140 - protein, 95 aa, Artificial Sequence
  Synthetic: ATI_1420_C02 w/ N leader and C tail
GVSDVPRDLEVVAATPTSLLISWRIKSYYAYRITYGETGGNSPVQEFTVRQHVATISGLKPGVDYTITVYARLGDVELVYEISINYRTEIDKPSQ

SEQ ID NO: 141 - protein, 101 aa, Artificial Sequence
  Synthetic: ATI_1420_C02 w/ N leader and C tail + his tag
GVSDVPRDLEVVAATPTSLLISWRIKSYYAYRITYGETGGNSPVQEFTVRQHVATISGLKPGVDYTITVYARLGDVELVYEISINYRTEIDKPSQHHHHHH

SEQ ID NO: 142 - protein, 90 aa, Artificial Sequence
  Synthetic: ATI_1420_C02 w/ N leader and modified C-terminus including PC
GVSDVPRDLEVVAATPTSLLISWRIKSYYAYRITYGETGGNSPVQEFTVRQHVATISGLKPGVDYTITVYARLGDVELVYEISINYRTPC

SEQ ID NO: 143 - protein, 93 aa, Artificial Sequence; identical to SEQ ID NO: 132
  Synthetic: ATI_1420_C02 w/ N leader and modified C-terminus including PC + his tag

SEQ ID NO: 144 - protein, 102 aa, Artificial Sequence
  Synthetic: ATI_1420_C02 full length
MGVSDVPRDLEVVAATPTSLLISWRIKSYYAYRITYGETGGNSPVQEFTVRQHVATISGLKPGVDYTITVYARLGDVELVYEISINYRTEIDKPSQHHHHHH

SEQ ID NO: 145 - protein, 80 aa, Artificial Sequence
  Synthetic: ATI_1420_C11 core
EVVAATPTSLLISWMYPLKSVPYRITYGETGGNSPVQEFTVYSSGATISGLKPGVDYTITVYAMSYSTYHAFMISINYRT

SEQ ID NO: 146 - protein, 8 aa, Artificial Sequence
  Synthetic: ATI_1420_C11 BC loop
MYPLKSVP

SEQ ID NO: 147 - protein, 4 aa, Artificial Sequence
  Synthetic: ATI_1420_C11 DE loop
YSSG

SEQ ID NO: 148 - protein, 10 aa, Artificial Sequence
  Synthetic: ATI_1420_C11 FG loop
MSYSTYHAFM

SEQ ID NO: 149 - protein, 89 aa, Artificial Sequence
  Synthetic: ATI_1420_C11 w/ N leader
GVSDVPRDLEVVAATPTSLLISWMYPLKSVPYRITYGETGGNSPVQEFTVYSSGATISGLKPGVDYTITVYAMSYSTYHAFMISINYRT

SEQ ID NO: 150 - protein, 95 aa, Artificial Sequence
  Synthetic: ATI_1420_C11 w/ N leader + his tag
GVSDVPRDLEVVAATPTSLLISWMYPLKSVPYRITYGETGGNSPVQEFTVYSSGATISGLKPGVDYTITVYAMSYSTYHAFMISINYRTHHHHHH

SEQ ID NO: 151 - protein, 96 aa, Artificial Sequence
  Synthetic: ATI_1420_C11 w/ N leader and C tail
GVSDVPRDLEVVAATPTSLLISWMYPLKSVPYRITYGETGGNSPVQEFTVYSSGATISGLKPGVDYTITVYAMSYSTYHAFMISINYRTEIDKPSQ

SEQ ID NO: 152 - protein, 102 aa, Artificial Sequence
  Synthetic: ATI_1420_C11 w/ N leader and C tail + his tag
GVSDVPRDLEVVAATPTSLLISWMYPLKSVPYRITYGETGGNSPVQEFTVYSSGATISGLKPGVDYTITVYAMSYSTYHAFMISINYRTEIDKPSQHHHHHH

SEQ ID NO: 153 - protein, 91 aa, Artificial Sequence
  Synthetic: ATI_1420_C11 w/ N leader and modified C-terminus including PC
GVSDVPRDLEVVAATPTSLLISWMYPLKSVPYRITYGETGGNSPVQEFTVYSSGATISGLKPGVDYTITVYAMSYSTYHAFMISINYRTPC

SEQ ID NO: 154 - protein, 97 aa, Artificial Sequence
  Synthetic: ATI_1420_C11 w/ N leader and modified C-terminus including PC + his tag
GVSDVPRDLEVVAATPTSLLISWMYPLKSVPYRITYGETGGNSPVQEFTVYSSGATISGLKPGVDYTITVYAMSYSTYHAFMISINYRTPCHHHHHH

SEQ ID NO: 155 - protein, 103 aa, Artificial Sequence
  Synthetic: AATI_1420_C11 full length
MGVSDVPRDLEVVAATPTSLLISWMYPLKSVPYRITYGETGGNSPVQEFTVYSSGATISGLKPGVDYTITVYAMSYSTYHAFMISINYRTEIDKPSQHHHHHH

SEQ ID NO: 156 - protein, 79 aa, Artificial Sequence
  Synthetic: ATI_1420_D01 core
EVVAATPTSLLISWRTVPETDYRITYGETGGNSPVQEFTVPDNTATISGLKPGVDYTITVYALETAHYNRDYISINYRT

SEQ ID NO: 157 - protein, 7 aa, Artificial Sequence
  Synthetic: ATI_1420_D01 BC loop
RTVPETD

SEQ ID NO: 158 - protein, 4 aa, Artificial Sequence
  Synthetic: ATI_1420_D01 DE loop
PDNT

SEQ ID NO: 159 - protein, 10 aa, Artificial Sequence
  Synthetic: ATI_1420_D01 FG loop
LETAHYNRDY

SEQ ID NO: 160 - protein, 88 aa, Artificial Sequence
  Synthetic: ATI_1420_D01 w/ N leader
GVSDVPRDLEVVAATPTSLLISWRTVPETDYRITYGETGGNSPVQEFTVPDNTATISGLKPGVDYTITVYALETAHYNRDYISINYRT

SEQ ID NO: 161 - protein, 94 aa, Artificial Sequence
  Synthetic: ATI_1420_D01 w/ N leader + his tag
GVSDVPRDLEVVAATPTSLLISWRTVPETDYRITYGETGGNSPVQEFTVPDNTATISGLKPGVDYTITVYALETAHYNRDYISINYRTHHHHHH

SEQ ID NO: 162 - protein, 95 aa, Artificial Sequence
  Synthetic: ATI_1420_D01 w/ N leader and C tail
GVSDVPRDLEVVAATPTSLLISWRTVPETDYRITYGETGGNSPVQEFTVPDNTATISGLKPGVDYTITVYALETAHYNRDYISINYRTEIDKPSQ

SEQ ID NO: 163 - protein, 101 aa, Artificial Sequence
  Synthetic: ATI_1420_D01 w/ N leader and C tail + his tag
GVSDVPRDLEVVAATPTSLLISWRTVPETDYRITYGETGGNSPVQEFTVPDNTATISGLKPGVDYTITVYALETAHYNRDYISINYRTEIDKPSQHHHHHH

SEQ ID NO: 164 - protein, 90 aa, Artificial Sequence
  Synthetic: ATI_1420_D01 w/ N leader and modified C-terminus including PC
GVSDVPRDLEVVAATPTSLLISWRTVPETDYRITYGETGGNSPVQEFTVPDNTATISGLKPGVDYTITVYALETAHYNRDYISINYRTPC

SEQ ID NO: 165 - protein, 96 aa, Artificial Sequence
  Synthetic: ATI_1420_D01 w/ N leader and modified C-terminus including PC + his tag
GVSDVPRDLEVVAATPTSLLISWRTVPETDYRITYGETGGNSPVQEFTVPDNTATISGLKPGVDYTITVYALETAHYNRDYISINYRTPCHHHHHH

SEQ ID NO: 166 - protein, 102 aa, Artificial Sequence
  Synthetic: ATI_1420_D01 full length
MGVSDVPRDLEVVAATPTSLLISWRTVPETDYRITYGETGGNSPVQEFTVPDNTATISGLKPGVDYTITVYALETAHYNRDYISINYRTEIDKPSQHHHHHH

SEQ ID NO: 167 - protein, 82 aa, Artificial Sequence
  Synthetic: ATI_1420_D05 core
EVVAATPTSLLISWTAYYSTIKYRITYGETGGNSPVQEFTVGPKHHATISGLKPGVDYTITVYAYNTKPGYHAHQISINYRT

SEQ ID NO: 168 - protein, 8 aa, Artificial Sequence
  Synthetic: ATI_1420_D05 BC loop
TAYYSTIK

SEQ ID NO: 169 - protein, 5 aa, Artificial Sequence
  Synthetic: ATI_1420_D05 DE loop
GPKHH

SEQ ID NO: 170 - protein, 11 aa, Artificial Sequence
  Synthetic: ATI_1420_D05 FG loop
YNTKPGYHAHQ

SEQ ID NO: 171 - protein, 91 aa, Artificial Sequence
  Synthetic: ATI_1420_D05 w/ N leader
GVSDVPRDLEVVAATPTSLLISWTAYYSTIKYRITYGETGGNSPVQEFTVGPKHHATISGLKPGVDYTITVYAYNTKPGYHAHQISINYRT

SEQ ID NO: 172 - protein, 97 aa, Artificial Sequence
  Synthetic: ATI_1420_D05 w/ N leader + his tag
GVSDVPRDLEVVAATPTSLLISWTAYYSTIKYRITYGETGGNSPVQEFTVGPKHHATISGLKPGVDYTITVYAYNTKPGYHAHQISINYRTHHHHHH

SEQ ID NO: 173 - protein, 98 aa, Artificial Sequence
  Synthetic: ATI_1420_D05 w/ N leader and C tail
GVSDVPRDLEVVAATPTSLLISWTAYYSTIKYRITYGETGGNSPVQEFTVGPKHHATISGLKPGVDYTITVYAYNTKPGYHAHQISINYRTEIDKPSQ

SEQ ID NO: 174 - protein, 104 aa, Artificial Sequence
  Synthetic: ATI_1420_D05 w/ N leader and C tail + his tag
GVSDVPRDLEVVAATPTSLLISWTAYYSTIKYRITYGETGGNSPVQEFTVGPKHHATISGLKPGVDYTITVYAYNTKPGYHAHQISINYRTEIDKPSQHHHHHH

SEQ ID NO: 175 - protein, 93 aa, Artificial Sequence
  Synthetic: ATI_1420_D05 w/ N leader and modified C-terminus including PC
GVSDVPRDLEVVAATPTSLLISWTAYYSTIKYRITYGETGGNSPVQEFTVGPKHHATISGLKPGVDYTITVYAYNTKPGYHAHQISINYRTPC

SEQ ID NO: 176 - protein, 99 aa, Artificial Sequence
  Synthetic: ATI_1420_D05 w/ N leader and modified C-terminus including PC + his tag
GVSDVPRDLEVVAATPTSLLISWTAYYSTIKYRITYGETGGNSPVQEFTVGPKHHATISGLKPGVDYTITVYAYNTKPGYHAHQISINYRTPCHHHHHH

SEQ ID NO: 177 - protein, 105 aa, Artificial Sequence
  Synthetic: ATI_1420_D05 full length
MGVSDVPRDLEVVAATPTSLLISWTAYYSTIKYRITYGETGGNSPVQEFTVGPKHHATISGLKPGVDYTITVYAYNTKPGYHAHQISINYRTEIDKPSQHHHHHH

SEQ ID NO: 178 - protein, 80 aa, Artificial Sequence
  Synthetic: ATI_1420_D10  core
EVVAATPTSLLISWRIPSYHIQYRITYGETGGNSPVQEFTVYQKYATISGLKPGVDYTITVYAVSPPKQLRFGISINYRT

SEQ ID NO: 179 - protein, 8 aa, Artificial Sequence
  Synthetic: ATI_1420_D10  BC loop
RIPSYHIQ

SEQ ID NO: 180 - protein, 4 aa, Artificial Sequence
  Synthetic: ATI_1420_D10  DE loop
YQKY

SEQ ID NO: 181 - protein, 10 aa, Artificial Sequence
  Synthetic: ATI_1420_D10  FG loop
VSPPKQLRFG

SEQ ID NO: 182 - protein, 89 aa, Artificial Sequence
  Synthetic: ATI_1420_D10  w/ N leader
GVSDVPRDLEVVAATPTSLLISWRIPSYHIQYRITYGETGGNSPVQEFTVYQKYATISGLKPGVDYTITVYAVSPPKQLRFGISINYRT

SEQ ID NO: 183 - protein, 95 aa, Artificial Sequence
  Synthetic: ATI_1420_D10  w/ N leader + his tag
GVSDVPRDLEVVAATPTSLLISWRIPSYHIQYRITYGETGGNSPVQEFTVYQKYATISGLKPGVDYTITVYAVSPPKQLRFGISINYRTHHHHHH

SEQ ID NO: 184 - protein, 96 aa, Artificial Sequence
  Synthetic: ATI_1420_D10  w/ N leader and C tail
GVSDVPRDLEVVAATPTSLLISWRIPSYHIQYRITYGETGGNSPVQEFTVYQKYATISGLKPGVDYTITVYAVSPPKQLRFGISINYRTEIDKPSQ

SEQ ID NO: 185 - protein, 102 aa, Artificial Sequence
  Synthetic: ATI_1420_D10  w/ N leader and C tail + his tag
GVSDVPRDLEVVAATPTSLLISWRIPSYHIQYRITYGETGGNSPVQEFTVYQKYATISGLKPGVDYTITVYAVSPPKQLRFGISINYRTEIDKPSQHHHHHH

SEQ ID NO: 186 - protein, 91 aa, Artificial Sequence
  Synthetic: ATI_1420_D10  w/ N leader and modified C-terminus including PC
GVSDVPRDLEVVAATPTSLLISWRIPSYHIQYRITYGETGGNSPVQEFTVYQKYATISGLKPGVDYTITVYAVSPPKQLRFGISINYRTPC

SEQ ID NO: 187 - protein, 97 aa, Artificial Sequence
  Synthetic: ATI_1420_D10  w/ N leader and modified C-terminus including PC + his tag
GVSDVPRDLEVVAATPTSLLISWRIPSYHIQYRITYGETGGNSPVQEFTVYQKYATISGLKPGVDYTITVYAVSPPKQLRFGISINYRTPCHHHHHH

SEQ ID NO: 188 - protein, 103 aa, Artificial Sequence
  Synthetic: ATI_1420_D010 full length
MGVSDVPRDLEVVAATPTSLLISWRIPSYHIQYRITYGETGGNSPVQEFTVYQKYATISGLKPGVDYTITVYAVSPPKQLRFGISINYRTEIDKPSQHHHHHH

SEQ ID NO: 189 - protein, 76 aa, Artificial Sequence
  Synthetic: ATI_1420_F10_core
EVVAATPTSLLISWPAPPSYVFYRITYGETGGNSPVQEFTVYPYMATISGLKPGVDYTITVYAYTSGFSISINYRT

SEQ ID NO: 190 - protein, 8 aa, Artificial Sequence
  Synthetic: ATI_1420_F10  BC loop
PAPPSYVF

SEQ ID NO: 191 - protein, 4 aa, Artificial Sequence
  Synthetic: ATI_1420_F10 DE loop
YPYM

SEQ ID NO: 192 - protein, 6 aa, Artificial Sequence
  Synthetic: ATI_1420_F10 FG loop
YTSGFS

SEQ ID NO: 193 - protein, 85 aa, Artificial Sequence
  Synthetic: ATI_1420_F10 w/ N leader
GVSDVPRDLEVVAATPTSLLISWPAPPSYVFYRITYGETGGNSPVQEFTVYPYMATISGLKPGVDYTITVYAYTSGFSISINYRT

SEQ ID NO: 194 - protein, 91 aa, Artificial Sequence
  Synthetic: ATI_1420_F10  w/ N leader + his tag
GVSDVPRDLEVVAATPTSLLISWPAPPSYVFYRITYGETGGNSPVQEFTVYPYMATISGLKPGVDYTITVYAYTSGFSISINYRTHHHHHH

SEQ ID NO: 195 - protein, 92 aa, Artificial Sequence
  Synthetic: ATI_1420_F10 w/ N leader and C tail
GVSDVPRDLEVVAATPTSLLISWPAPPSYVFYRITYGETGGNSPVQEFTVYPYMATISGLKPGVDYTITVYAYTSGFSISINYRTEIDKPSQ

SEQ ID NO: 196 - protein, 98 aa, Artificial Sequence
  Synthetic: ATI_1420_F10  w/ N leader and C tail + his tag
GVSDVPRDLEVVAATPTSLLISWPAPPSYVFYRITYGETGGNSPVQEFTVYPYMATISGLKPGVDYTITVYAYTSGFSISINYRTEIDKPSQHHHHHH

SEQ ID NO: 197 - protein, 87 aa, Artificial Sequence
  Synthetic: ATI_1420_F10  w/ N leader and modified C-terminus including PC
GVSDVPRDLEVVAATPTSLLISWPAPPSYVFYRITYGETGGNSPVQEFTVYPYMATISGLKPGVDYTITVYAYTSGFSISINYRTPC

SEQ ID NO: 198 - protein, 93 aa, Artificial Sequence
  Synthetic: ATI_1420_F10  w/ N leader and modified C-terminus including PC + his tag
GVSDVPRDLEVVAATPTSLLISWPAPPSYVFYRITYGETGGNSPVQEFTVYPYMATISGLKPGVDYTITVYAYTSGFSISINYRTPCHHHHHH

SEQ ID NO: 199 - protein, 99 aa, Artificial Sequence
  Synthetic: ATI_1420_F10 full length
MGVSDVPRDLEVVAATPTSLLISWPAPPSYVFYRITYGETGGNSPVQEFTVYPYMATISGLKPGVDYTITVYAYTSGFSISINYRTEIDKPSQHHHHHH

SEQ ID NO: 200 - protein, 79 aa, Artificial Sequence
  Synthetic: ATI_1421_C05_core
EVVAATPTSLLISWYMDHKSKYRITYGETGGNSPVQEFTVPDQRATISGLKPGVDYTITVYALSEAHYLRDKISINYRT

SEQ ID NO: 201 - protein, 7 aa, Artificial Sequence
  Synthetic: ATI_1421_C05  BC loop
YMDHKSK

SEQ ID NO: 202 - protein, 4 aa, Artificial Sequence
  Synthetic: ATI_1421_C05 DE loop
PDQR

SEQ ID NO: 203 - protein, 10 aa, Artificial Sequence
  Synthetic: ATI_1421_C05 FG loop
LSEAHYLRDK

SEQ ID NO: 204 - protein, 88 aa, Artificial Sequence
  Synthetic: ATI_1421_C05 w/ N leader
GVSDVPRDLEVVAATPTSLLISWYMDHKSKYRITYGETGGNSPVQEFTVPDQRATISGLKPGVDYTITVYALSEAHYLRDKISINYRT

SEQ ID NO: 205 - protein, 94 aa, Artificial Sequence
  Synthetic: ATI_1421_C05  w/ N leader + his tag
GVSDVPRDLEVVAATPTSLLISWYMDHKSKYRITYGETGGNSPVQEFTVPDQRATISGLKPGVDYTITVYALSEAHYLRDKISINYRTHHHHHH

SEQ ID NO: 206 - protein, 95 aa, Artificial Sequence
  Synthetic: ATI_1421_C05 w/ N leader and C tail
GVSDVPRDLEVVAATPTSLLISWYMDHKSKYRITYGETGGNSPVQEFTVPDQRATISGLKPGVDYTITVYALSEAHYLRDKISINYRTEIDKPSQ

SEQ ID NO: 207 - protein, 101 aa, Artificial Sequence
  Synthetic: ATI_1421_C05  w/ N leader and C tail + his tag
GVSDVPRDLEVVAATPTSLLISWYMDHKSKYRITYGETGGNSPVQEFTVPDQRATISGLKPGVDYTITVYALSEAHYLRDKISINYRTEIDKPSQHHHHHH

SEQ ID NO: 208 - protein, 90 aa, Artificial Sequence
  Synthetic: ATI_1421_C05  w/ N leader and modified C-terminus including PC
GVSDVPRDLEVVAATPTSLLISWYMDHKSKYRITYGETGGNSPVQEFTVPDQRATISGLKPGVDYTITVYALSEAHYLRDKISINYRTPC

SEQ ID NO: 209 - protein, 96 aa, Artificial Sequence
  Synthetic: ATI_1421_C05 w/ N leader and modified C-terminus including PC + his tag
GVSDVPRDLEVVAATPTSLLISWYMDHKSKYRITYGETGGNSPVQEFTVPDQRATISGLKPGVDYTITVYALSEAHYLRDKISINYRTPCHHHHHH

SEQ ID NO: 210 - protein, 102 aa, Artificial Sequence
  Synthetic: ATI_1421_C05 full length
MGVSDVPRDLEVVAATPTSLLISWYMDHKSKYRITYGETGGNSPVQEFTVPDQRATISGLKPGVDYTITVYALSEAHYLRDKISINYRTEIDKPSQHHHHHH

SEQ ID NO: 211 - protein, 79 aa, Artificial Sequence
  Synthetic: ATI_1421_C06 core
EVVAATPTSLLISWENLASYQYRITYGETGGNSPVQEFTVPDQAATISGLKPGVDYTITVYALQTAHYYRQHISINYRT

SEQ ID NO: 212 - protein, 7 aa, Artificial Sequence
  Synthetic: ATI_1421_C06 BC loop
ENLASYQ

SEQ ID NO: 213 - protein, 4 aa, Artificial Sequence
  Synthetic: ATI_1421_C06DE loop
PDQA

SEQ ID NO: 214 - protein, 10 aa, Artificial Sequence
  Synthetic: ATI_1421_C06FG loop
LQTAHYYRQH

SEQ ID NO: 215 - protein, 88 aa, Artificial Sequence
  Synthetic: ATI_1421_C06 w/ N leader
GVSDVPRDLEVVAATPTSLLISWENLASYQYRITYGETGGNSPVQEFTVPDQAATISGLKPGVDYTITVYALQTAHYYRQHISINYRT

SEQ ID NO: 216 - protein, 94 aa, Artificial Sequence
  Synthetic: ATI_1421_C06 w/ N leader + his tag
GVSDVPRDLEVVAATPTSLLISWENLASYQYRITYGETGGNSPVQEFTVPDQAATISGLKPGVDYTITVYALQTAHYYRQHISINYRTHHHHHH

SEQ ID NO: 217 - protein, 95 aa, Artificial Sequence
  Synthetic: ATI_1421_C06w/ N leader and C tail
GVSDVPRDLEVVAATPTSLLISWENLASYQYRITYGETGGNSPVQEFTVPDQAATISGLKPGVDYTITVYALQTAHYYRQHISINYRTEIDKPSQ

SEQ ID NO: 218 - protein, 101 aa, Artificial Sequence
  Synthetic: ATI_1421_C06 w/ N leader and C tail + his tag
GVSDVPRDLEVVAATPTSLLISWENLASYQYRITYGETGGNSPVQEFTVPDQAATISGLKPGVDYTITVYALQTAHYYRQHISINYRTEIDKPSQHHHHHH

SEQ ID NO: 219 - protein, 90 aa, Artificial Sequence
  Synthetic: ATI_1421_C06 w/ N leader and modified C-terminus including PC
GVSDVPRDLEVVAATPTSLLISWENLASYQYRITYGETGGNSPVQEFTVPDQAATISGLKPGVDYTITVYALQTAHYYRQHISINYRTPC

SEQ ID NO: 220 - protein, 96 aa, Artificial Sequence
  Synthetic: ATI_1421_C06 w/ N leader and modified C-terminus including PC + his tag
GVSDVPRDLEVVAATPTSLLISWENLASYQYRITYGETGGNSPVQEFTVPDQAATISGLKPGVDYTITVYALQTAHYYRQHISINYRTPCHHHHHH

SEQ ID NO: 221 - protein, 102 aa, Artificial Sequence
  Synthetic: ATI_1421_C06 full length
MGVSDVPRDLEVVAATPTSLLISWENLASYQYRITYGETGGNSPVQEFTVPDQAATISGLKPGVDYTITVYALQTAHYYRQHISINYRTEIDKPSQHHHHHH

SEQ ID NO: 222 - protein, 79 aa, Artificial Sequence
  Synthetic: ATI 1421_D05 core
EVVAATPTSLLISWYYVQYNDYRITYGETGGNSPVQEFTVPDQSATISGLKPGVDYTITVYALEKAHYYRQNISINYRT

SEQ ID NO: 223 - protein, 7 aa, Artificial Sequence
  Synthetic: ATI 1421_D05 BC loop
YYVQYND

SEQ ID NO: 224 - protein, 4 aa, Artificial Sequence
  Synthetic: ATI 1421_D05 DE loop
PDQS

SEQ ID NO: 225 - protein, 10 aa, Artificial Sequence
  Synthetic: ATI 1421_D05 FG loop
LEKAHYYRQN

SEQ ID NO: 226 - protein, 88 aa, Artificial Sequence
  Synthetic: ATI 1421_D05 w/ N leader
GVSDVPRDLEVVAATPTSLLISWYYVQYNDYRITYGETGGNSPVQEFTVPDQSATISGLKPGVDYTITVYALEKAHYYRQNISINYRT

SEQ ID NO: 227 - protein, 94 aa, Artificial Sequence
  Synthetic: ATI 1421_D05 w/ N leader + his tag
GVSDVPRDLEVVAATPTSLLISWYYVQYNDYRITYGETGGNSPVQEFTVPDQSATISGLKPGVDYTITVYALEKAHYYRQNISINYRTHHHHHH

SEQ ID NO: 228 - protein, 95 aa, Artificial Sequence
  Synthetic: ATI 1421_D05 w/ N leader and C tail
GVSDVPRDLEVVAATPTSLLISWYYVQYNDYRITYGETGGNSPVQEFTVPDQSATISGLKPGVDYTITVYALEKAHYYRQNISINYRTEIDKPSQ

SEQ ID NO: 229 - protein, 101 aa, Artificial Sequence
  Synthetic: ATI 1421_D05 w/ N leader and C tail + his tag
GVSDVPRDLEVVAATPTSLLISWYYVQYNDYRITYGETGGNSPVQEFTVPDQSATISGLKPGVDYTITVYALEKAHYYRQNISINYRTEIDKPSQHHHHHH

SEQ ID NO: 230 - protein, 90 aa, Artificial Sequence
  Synthetic: ATI 1421_D05 w/ N leader and modified C-terminus including PC
GVSDVPRDLEVVAATPTSLLISWYYVQYNDYRITYGETGGNSPVQEFTVPDQSATISGLKPGVDYTITVYALEKAHYYRQNISINYRTPC

SEQ ID NO: 231 - protein, 96 aa, Artificial Sequence
  Synthetic: ATI 1421_D05 w/ N leader and modified C-terminus including PC + his tag
GVSDVPRDLEVVAATPTSLLISWYYVQYNDYRITYGETGGNSPVQEFTVPDQSATISGLKPGVDYTITVYALEKAHYYRQNISINYRTPCHHHHHH

SEQ ID NO: 232 - protein, 102 aa, Artificial Sequence
  Synthetic: ATI 1421_D05  full length
MGVSDVPRDLEVVAATPTSLLISWYYVQYNDYRITYGETGGNSPVQEFTVPDQSATISGLKPGVDYTITVYALEKAHYYRQNISINYRTEIDKPSQHHHHHH

SEQ ID NO: 233 - protein, 79 aa, Artificial Sequence
  Synthetic: ATI_1421_D06 core
EVVAATPTSLLISWGHNYDDEYRITYGETGGNSPVQEFTVPDQYATISGLKPGVDYTITVYALAEAHVRKNHISINYRT

SEQ ID NO: 234 - protein, 7 aa, Artificial Sequence
  Synthetic: ATI_1421_D06 BC loop
GHNYDDE

SEQ ID NO: 235 - protein, 4 aa, Artificial Sequence
  Synthetic: ATI_1421_D06  DE loop
PDQY

SEQ ID NO: 236 - protein, 10 aa, Artificial Sequence
  Synthetic: ATI_1421_D06  FG loop
LAEAHVRKNH

SEQ ID NO: 237 - protein, 88 aa, Artificial Sequence
  Synthetic: ATI_1421_D06 w/ N leader
GVSDVPRDLEVVAATPTSLLISWGHNYDDEYRITYGETGGNSPVQEFTVPDQYATISGLKPGVDYTITVYALAEAHVRKNHISINYRT

SEQ ID NO: 238 - protein, 94 aa, Artificial Sequence
  Synthetic: ATI_1421_D06 w/ N leader + his tag
GVSDVPRDLEVVAATPTSLLISWGHNYDDEYRITYGETGGNSPVQEFTVPDQYATISGLKPGVDYTITVYALAEAHVRKNHISINYRTHHHHHH

SEQ ID NO: 239 - protein, 95 aa, Artificial Sequence
  Synthetic: ATI_1421_D06 w/ N leader and C tail
GVSDVPRDLEVVAATPTSLLISWGHNYDDEYRITYGETGGNSPVQEFTVPDQYATISGLKPGVDYTITVYALAEAHVRKNHISINYRTEIDKPSQ

SEQ ID NO: 240 - protein, 101 aa, Artificial Sequence
  Synthetic: ATI_1421_D06 w/ N leader and C tail + his tag
GVSDVPRDLEVVAATPTSLLISWGHNYDDEYRITYGETGGNSPVQEFTVPDQYATISGLKPGVDYTITVYALAEAHVRKNHISINYRTEIDKPSQHHHHHH

SEQ ID NO: 241 - protein, 90 aa, Artificial Sequence
  Synthetic: ATI_1421_D06 w/ N leader and modified C-terminus including PC
GVSDVPRDLEVVAATPTSLLISWGHNYDDEYRITYGETGGNSPVQEFTVPDQYATISGLKPGVDYTITVYALAEAHVRKNHISINYRTPC

SEQ ID NO: 242 - protein, 96 aa, Artificial Sequence
  Synthetic: ATI_1421_D06 w/ N leader and modified C-terminus including PC + his tag
GVSDVPRDLEVVAATPTSLLISWGHNYDDEYRITYGETGGNSPVQEFTVPDQYATISGLKPGVDYTITVYALAEAHVRKNHISINYRTPCHHHHHH

SEQ ID NO: 243 - protein, 102 aa, Artificial Sequence
  Synthetic: ATI_1421_D06  full length
MGVSDVPRDLEVVAATPTSLLISWGHNYDDEYRITYGETGGNSPVQEFTVPDQYATISGLKPGVDYTITVYALAEAHVRKNHISINYRTEIDKPSQHHHHHH

SEQ ID NO: 244 - protein, 79 aa, Artificial Sequence
  Synthetic: ATI_1421_E03 core
EVVAATPTSLLISWVYHYDAQYRITYGETGGNSPVQEFTVPDQKATISGLKPGVDYTITVYALSEAHHKRDSISINYRT

SEQ ID NO: 245 - protein, 7 aa, Artificial Sequence
  Synthetic: ATI_1421_E03 BC loop
VYHYDAQ

SEQ ID NO: 246 - protein, 4 aa, Artificial Sequence
  Synthetic: ATI_1421_E03 DE loop
PDQK

SEQ ID NO: 247 - protein, 10 aa, Artificial Sequence
  Synthetic: ATI_1421_E03 FG loop
LSEAHHKRDS

SEQ ID NO: 248 - protein, 94 aa, Artificial Sequence
  Synthetic: ATI_1421_E03 w/ N leader
GVSDVPRDLEVVAATPTSLLISWVYHYDAQYRITYGETGGNSPVQEFTVPDQKATISGLKPGVDYTITVYALSEAHHKRDSISINYRTHHHHHH

SEQ ID NO: 249 - protein, 95 aa, Artificial Sequence
  Synthetic: ATI_1421_E03w/ N leader + his tag
GVSDVPRDLEVVAATPTSLLISWVYHYDAQYRITYGETGGNSPVQEFTVPDQKATISGLKPGVDYTITVYALSEAHHKRDSISINYRTEIDKPSQ

SEQ ID NO: 250 - protein, 101 aa, Artificial Sequence
  Synthetic: ATI_1421_E03w/ N leader and C tail
GVSDVPRDLEVVAATPTSLLISWVYHYDAQYRITYGETGGNSPVQEFTVPDQKATISGLKPGVDYTITVYALSEAHHKRDSISINYRTEIDKPSQHHHHHH

SEQ ID NO: 251 - protein, 90 aa, Artificial Sequence
  Synthetic: ATI_1421_E03 w/ N leader and C tail + his tag
GVSDVPRDLEVVAATPTSLLISWVYHYDAQYRITYGETGGNSPVQEFTVPDQKATISGLKPGVDYTITVYALSEAHHKRDSISINYRTPC

SEQ ID NO: 252 - protein, 96 aa, Artificial Sequence
  Synthetic: ATI_1421_E03 w/ N leader and modified C-terminus including PC
GVSDVPRDLEVVAATPTSLLISWVYHYDAQYRITYGETGGNSPVQEFTVPDQKATISGLKPGVDYTITVYALSEAHHKRDSISINYRTPCHHHHHH

SEQ ID NO: 253 - protein, 88 aa, Artificial Sequence
  Synthetic: ATI_1421_E03 w/ N leader and modified C-terminus including PC + his tag
GVSDVPRDLEVVAATPTSLLISWVYHYDAQYRITYGETGGNSPVQEFTVPDQKATISGLKPGVDYTITVYALSEAHHKRDSISINYRT

SEQ ID NO: 254 - protein, 102 aa, Artificial Sequence
  Synthetic: ATI_1421_E03  full length
MGVSDVPRDLEVVAATPTSLLISWVYHYDAQYRITYGETGGNSPVQEFTVPDQKATISGLKPGVDYTITVYALSEAHHKRDSISINYRTEIDKPSQHHHHHH

SEQ ID NO: 255 - protein, 79 aa, Artificial Sequence
  Synthetic: ATI_1421_E04 core
EVVAATPTSLLISWSYNGPIEYRITYGETGGNSPVQEFTVPDQQATISGLKPGVDYTITVYALEEAHYSRQSISINYRT

SEQ ID NO: 256 - protein, 7 aa, Artificial Sequence
  Synthetic: ATI_1421_E04 BC loop
SYNGPIE

SEQ ID NO: 257 - protein, 4 aa, Artificial Sequence
  Synthetic: ATI_1421_E04 DE loop
PDQQ

SEQ ID NO: 258 - protein, 10 aa, Artificial Sequence
  Synthetic: ATI_1421_E04 FG loop
LEEAHYSRQS

SEQ ID NO: 259 - protein, 88 aa, Artificial Sequence
  Synthetic: ATI_1421_E04 w/ N leader
GVSDVPRDLEVVAATPTSLLISWSYNGPIEYRITYGETGGNSPVQEFTVPDQQATISGLKPGVDYTITVYALEEAHYSRQSISINYRT

SEQ ID NO: 260 - protein, 94 aa, Artificial Sequence
  Synthetic: ATI_1421_E04 w/ N leader + his tag
GVSDVPRDLEVVAATPTSLLISWSYNGPIEYRITYGETGGNSPVQEFTVPDQQATISGLKPGVDYTITVYALEEAHYSRQSISINYRTHHHHHH

SEQ ID NO: 261 - protein, 95 aa, Artificial Sequence
  Synthetic: ATI_1421_E04 w/ N leader and C tail
GVSDVPRDLEVVAATPTSLLISWSYNGPIEYRITYGETGGNSPVQEFTVPDQQATISGLKPGVDYTITVYALEEAHYSRQSISINYRTEIDKPSQ

SEQ ID NO: 262 - protein, 101 aa, Artificial Sequence
  Synthetic: ATI_1421_E04 w/ N leader and C tail + his tag
GVSDVPRDLEVVAATPTSLLISWSYNGPIEYRITYGETGGNSPVQEFTVPDQQATISGLKPGVDYTITVYALEEAHYSRQSISINYRTEIDKPSQHHHHHH

SEQ ID NO: 263 - protein, 90 aa, Artificial Sequence
  Synthetic: ATI_1421_E04 w/ N leader and modified C-terminus including PC
GVSDVPRDLEVVAATPTSLLISWSYNGPIEYRITYGETGGNSPVQEFTVPDQQATISGLKPGVDYTITVYALEEAHYSRQSISINYRTPC

SEQ ID NO: 264 - protein, 96 aa, Artificial Sequence
  Synthetic: ATI_1421_E04 w/ N leader and modified C-terminus including PC + his tag
GVSDVPRDLEVVAATPTSLLISWSYNGPIEYRITYGETGGNSPVQEFTVPDQQATISGLKPGVDYTITVYALEEAHYSRQSISINYRTPCHHHHHH

SEQ ID NO: 265 - protein, 102 aa, Artificial Sequence
  Synthetic: ATI_1421_E04 full length
MGVSDVPRDLEVVAATPTSLLISWSYNGPIEYRITYGETGGNSPVQEFTVPDQQATISGLKPGVDYTITVYALEEAHYSRQSISINYRTEIDKPSQHHHHHH

SEQ ID NO: 266 - protein, 79 aa, Artificial Sequence
  Synthetic: ATI_1421_F03 core
EVVAATPTSLLISWISVQTYDYRITYGETGGNSPVQEFTVPDQSATISGLKPGVDYTITVYALEKAHYYRQNISINYRT

SEQ ID NO: 267 - protein, 7 aa, Artificial Sequence
  Synthetic: ATI_1421_F03 BC loop
ISVQTYD

SEQ ID NO: 268 - protein, 4 aa, Artificial Sequence
  Synthetic: ATI_1421_F03 DE loop
PDQS

SEQ ID NO: 269 - protein, 10 aa, Artificial Sequence
  Synthetic: ATI_1421_F03 FG loop
LEKAHYYRQN

SEQ ID NO: 270 - protein, 88 aa, Artificial Sequence
  Synthetic: ATI_1421_F03 w/ N leader
GVSDVPRDLEVVAATPTSLLISWISVQTYDYRITYGETGGNSPVQEFTVPDQSATISGLKPGVDYTITVYALEKAHYYRQNISINYRT

SEQ ID NO: 271 - protein, 94 aa, Artificial Sequence
  Synthetic: ATI_1421_F03 w/ N leader + his tag
GVSDVPRDLEVVAATPTSLLISWISVQTYDYRITYGETGGNSPVQEFTVPDQSATISGLKPGVDYTITVYALEKAHYYRQNISINYRTHHHHHH

SEQ ID NO: 272 - protein, 95 aa, Artificial Sequence
  Synthetic: ATI_1421_F03 w/ N leader and C tail
GVSDVPRDLEVVAATPTSLLISWISVQTYDYRITYGETGGNSPVQEFTVPDQSATISGLKPGVDYTITVYALEKAHYYRQNISINYRTEIDKPSQ

SEQ ID NO: 273 - protein, 101 aa, Artificial Sequence
  Synthetic: ATI_1421_F03 w/ N leader and C tail + his tag
GVSDVPRDLEVVAATPTSLLISWISVQTYDYRITYGETGGNSPVQEFTVPDQSATISGLKPGVDYTITVYALEKAHYYRQNISINYRTEIDKPSQHHHHHH

SEQ ID NO: 274 - protein, 90 aa, Artificial Sequence
  Synthetic: ATI_1421_F03 w/ N leader and modified C-terminus including PC
GVSDVPRDLEVVAATPTSLLISWISVQTYDYRITYGETGGNSPVQEFTVPDQSATISGLKPGVDYTITVYALEKAHYYRQNISINYRTPC

SEQ ID NO: 275 - protein, 96 aa, Artificial Sequence
  Synthetic: ATI_1421_F03 w/ N leader and modified C-terminus including PC + his tag
GVSDVPRDLEVVAATPTSLLISWISVQTYDYRITYGETGGNSPVQEFTVPDQSATISGLKPGVDYTITVYALEKAHYYRQNISINYRTPCHHHHHH

SEQ ID NO: 276 - protein, 102 aa, Artificial Sequence
  Synthetic: ATI_1421_F03 full length
MGVSDVPRDLEVVAATPTSLLISWISVQTYDYRITYGETGGNSPVQEFTVPDQSATISGLKPGVDYTITVYALEKAHYYRQNISINYRTEIDKPSQHHHHHH

SEQ ID NO: 277 - protein, 79 aa, Artificial Sequence
  Synthetic: ATI_1421_F05 core
EVVAATPTSLLISWLARHDARYRITYGETGGNSPVQEFTVPDRMATISGLKPGVDYTITVYALEQAHYYRLYISINYRT

SEQ ID NO: 278 - protein, 7 aa, Artificial Sequence
  Synthetic: ATI_1421_F05 BC loop
LARHDAR

SEQ ID NO: 279 - protein, 4 aa, Artificial Sequence
  Synthetic: ATI_1421_F05 DE loop
PDRM

SEQ ID NO: 280 - protein, 10 aa, Artificial Sequence
  Synthetic: ATI_1421_F05 FG loop
LEQAHYYRLY

SEQ ID NO: 281 - protein, 88 aa, Artificial Sequence
  Synthetic: ATI_1421_F05 w/ N leader
GVSDVPRDLEVVAATPTSLLISWLARHDARYRITYGETGGNSPVQEFTVPDRMATISGLKPGVDYTITVYALEQAHYYRLYISINYRT

SEQ ID NO: 282 - protein, 94 aa, Artificial Sequence
  Synthetic: ATI_1421_F05 w/ N leader + his tag
GVSDVPRDLEVVAATPTSLLISWLARHDARYRITYGETGGNSPVQEFTVPDRMATISGLKPGVDYTITVYALEQAHYYRLYISINYRTHHHHHH

SEQ ID NO: 283 - protein, 95 aa, Artificial Sequence
  Synthetic: ATI_1421_F05 w/ N leader and C tail
GVSDVPRDLEVVAATPTSLLISWLARHDARYRITYGETGGNSPVQEFTVPDRMATISGLKPGVDYTITVYALEQAHYYRLYISINYRTEIDKPSQ

SEQ ID NO: 284 - protein, 101 aa, Artificial Sequence
  Synthetic: ATI_1421_F05 w/ N leader and C tail + his tag
GVSDVPRDLEVVAATPTSLLISWLARHDARYRITYGETGGNSPVQEFTVPDRMATISGLKPGVDYTITVYALEQAHYYRLYISINYRTEIDKPSQHHHHHH

SEQ ID NO: 285 - protein, 90 aa, Artificial Sequence
  Synthetic: ATI_1421_F05 w/ N leader and modified C-terminus including PC
GVSDVPRDLEVVAATPTSLLISWLARHDARYRITYGETGGNSPVQEFTVPDRMATISGLKPGVDYTITVYALEQAHYYRLYISINYRTPC

SEQ ID NO: 286 - protein, 96 aa, Artificial Sequence
  Synthetic: ATI_1421_F05 w/ N leader and modified C-terminus including PC + his tag
GVSDVPRDLEVVAATPTSLLISWLARHDARYRITYGETGGNSPVQEFTVPDRMATISGLKPGVDYTITVYALEQAHYYRLYISINYRTPCHHHHHH

SEQ ID NO: 287 - protein, 102 aa, Artificial Sequence
  Synthetic: ATI_1421_F05 full length
MGVSDVPRDLEVVAATPTSLLISWLARHDARYRITYGETGGNSPVQEFTVPDRMATISGLKPGVDYTITVYALEQAHYYRLYISINYRTEIDKPSQHHHHHH

SEQ ID NO: 288 - protein, 82 aa, Artificial Sequence
  Synthetic: ATI_1421_G07 core
EVVAATPTSLLISWHSPTSGITYRITYGETGGNSPVQEFTVPYDPSATISGLKPGVDYTITVYAPYGSQYYPGYHISINYRT

SEQ ID NO: 289 - protein, 8 aa, Artificial Sequence
  Synthetic: ATI_1421_G07 BC loop
HSPTSGIT

SEQ ID NO: 290 - protein, 5 aa, Artificial Sequence
  Synthetic: ATI_1421_G07 DE loop
PYDPS

SEQ ID NO: 291 - protein, 11 aa, Artificial Sequence
  Synthetic: ATI_1421_G07 FG loop
PYGSQYYPGYH

SEQ ID NO: 292 - protein, 91 aa, Artificial Sequence
  Synthetic: ATI_1421_G07 w/ N leader
GVSDVPRDLEVVAATPTSLLISWHSPTSGITYRITYGETGGNSPVQEFTVPYDPSATISGLKPGVDYTITVYAPYGSQYYPGYHISINYRT

SEQ ID NO: 293 - protein, 97 aa, Artificial Sequence
  Synthetic: ATI_1421_G07 w/ N leader + his tag
GVSDVPRDLEVVAATPTSLLISWHSPTSGITYRITYGETGGNSPVQEFTVPYDPSATISGLKPGVDYTITVYAPYGSQYYPGYHISINYRTHHHHHH

SEQ ID NO: 294 - protein, 98 aa, Artificial Sequence
  Synthetic: ATI_1421_G07 w/ N leader and C tail
GVSDVPRDLEVVAATPTSLLISWHSPTSGITYRITYGETGGNSPVQEFTVPYDPSATISGLKPGVDYTITVYAPYGSQYYPGYHISINYRTEIDKPSQ

SEQ ID NO: 295 - protein, 104 aa, Artificial Sequence
  Synthetic: ATI_1421_G07 w/ N leader and C tail + his tag
GVSDVPRDLEVVAATPTSLLISWHSPTSGITYRITYGETGGNSPVQEFTVPYDPSATISGLKPGVDYTITVYAPYGSQYYPGYHISINYRTEIDKPSQHHHHHH

SEQ ID NO: 296 - protein, 93 aa, Artificial Sequence
  Synthetic: ATI_1421_G07 w/ N leader and modified C-terminus including PC
GVSDVPRDLEVVAATPTSLLISWHSPTSGITYRITYGETGGNSPVQEFTVPYDPSATISGLKPGVDYTITVYAPYGSQYYPGYHISINYRTPC

SEQ ID NO: 297 - protein, 99 aa, Artificial Sequence
  Synthetic: ATI_1421_G07 w/ N leader and modified C-terminus including PC + his tag
GVSDVPRDLEVVAATPTSLLISWHSPTSGITYRITYGETGGNSPVQEFTVPYDPSATISGLKPGVDYTITVYAPYGSQYYPGYHISINYRTPCHHHHHH

SEQ ID NO: 298 - protein, 105 aa, Artificial Sequence
  Synthetic: ATI_1421_G07 full length
MGVSDVPRDLEVVAATPTSLLISWHSPTSGITYRITYGETGGNSPVQEFTVPYDPSATISGLKPGVDYTITVYAPYGSQYYPGYHISINYRTEIDKPSQHHHHHH

SEQ ID NO: 299 - protein, 79 aa, Artificial Sequence
  Synthetic: ATI_1421_H03  core
EVVAATPTSLLISWVYHYDAQYRITYGETGGNSPVQEFTVPDSSATISGLKPGVDYTITVYALEQAHIDRTTISINYRT

SEQ ID NO: 300 - protein, 7 aa, Artificial Sequence
  Synthetic: ATI_1421_H03  BC loop
VYHYDAQ

SEQ ID NO: 301 - protein, 4 aa, Artificial Sequence
  Synthetic: ATI_1421_H03  DE loop
PDSS

SEQ ID NO: 302 - protein, 10 aa, Artificial Sequence
  Synthetic: ATI_1421_H03  FG loop
LEQAHIDRTT

SEQ ID NO: 303 - protein, 88 aa, Artificial Sequence
  Synthetic: ATI_1421_H03  w/ N leader
GVSDVPRDLEVVAATPTSLLISWVYHYDAQYRITYGETGGNSPVQEFTVPDSSATISGLKPGVDYTITVYALEQAHIDRTTISINYRT

SEQ ID NO: 304 - protein, 94 aa, Artificial Sequence
  Synthetic: ATI_1421_H03  w/ N leader + his tag
GVSDVPRDLEVVAATPTSLLISWVYHYDAQYRITYGETGGNSPVQEFTVPDSSATISGLKPGVDYTITVYALEQAHIDRTTISINYRTHHHHHH

SEQ ID NO: 305 - protein, 95 aa, Artificial Sequence
  Synthetic: ATI_1421_H03 w/ N leader and C tail
GVSDVPRDLEVVAATPTSLLISWVYHYDAQYRITYGETGGNSPVQEFTVPDSSATISGLKPGVDYTITVYALEQAHIDRTTISINYRTEIDKPSQ

SEQ ID NO: 306 - protein, 101 aa, Artificial Sequence
  Synthetic: ATI_1421_H03 w/ N leader and C tail + his tag
GVSDVPRDLEVVAATPTSLLISWVYHYDAQYRITYGETGGNSPVQEFTVPDSSATISGLKPGVDYTITVYALEQAHIDRTTISINYRTEIDKPSQHHHHHH

SEQ ID NO: 307 - protein, 90 aa, Artificial Sequence
  Synthetic: ATI_1421_H03 w/ N leader and modified C-terminus including PC
GVSDVPRDLEVVAATPTSLLISWVYHYDAQYRITYGETGGNSPVQEFTVPDSSATISGLKPGVDYTITVYALEQAHIDRTTISINYRTPC

SEQ ID NO: 308 - protein, 96 aa, Artificial Sequence
  Synthetic: ATI_1421_H03 w/ N leader and modified C-terminus including PC + his tag
GVSDVPRDLEVVAATPTSLLISWVYHYDAQYRITYGETGGNSPVQEFTVPDSSATISGLKPGVDYTITVYALEQAHIDRTTISINYRTPCHHHHHH

SEQ ID NO: 309 - protein, 102 aa, Artificial Sequence
  Synthetic: ATI_1421_H03  full length
MGVSDVPRDLEVVAATPTSLLISWVYHYDAQYRITYGETGGNSPVQEFTVPDSSATISGLKPGVDYTITVYALEQAHIDRTTISINYRTEIDKPSQHHHHHH

SEQ ID NO: 310 - protein, 79 aa, Artificial Sequence
  Synthetic: ATI_1421_H05 core
EVVAATPTSLLISWTSVLLKDYRITYGETGGNSPVQEFTVPDQHATISGLKPGVDYTITVYALQNAHHERLYISINYRT

SEQ ID NO: 311 - protein, 7 aa, Artificial Sequence
  Synthetic: ATI_1421_H05 BC loop
TSVLLKD

SEQ ID NO: 312 - protein, 4 aa, Artificial Sequence
  Synthetic: ATI_1421_H05 DE loop
PDQH

SEQ ID NO: 313 - protein, 10 aa, Artificial Sequence
  Synthetic: ATI_1421_H05 FG loop
LQNAHHERLY

SEQ ID NO: 314 - protein, 88 aa, Artificial Sequence
  Synthetic: ATI_1421_H05 w/ N leader
GVSDVPRDLEVVAATPTSLLISWTSVLLKDYRITYGETGGNSPVQEFTVPDQHATISGLKPGVDYTITVYALQNAHHERLYISINYRT

SEQ ID NO: 315 - protein, 94 aa, Artificial Sequence
  Synthetic: ATI_1421_H05 w/ N leader + his tag
GVSDVPRDLEVVAATPTSLLISWTSVLLKDYRITYGETGGNSPVQEFTVPDQHATISGLKPGVDYTITVYALQNAHHERLYISINYRTHHHHHH

SEQ ID NO: 316 - protein, 95 aa, Artificial Sequence
  Synthetic: ATI_1421_H05 w/ N leader and C tail
GVSDVPRDLEVVAATPTSLLISWTSVLLKDYRITYGETGGNSPVQEFTVPDQHATISGLKPGVDYTITVYALQNAHHERLYISINYRTEIDKPSQ

SEQ ID NO: 317 - protein, 101 aa, Artificial Sequence
  Synthetic: ATI_1421_H05 w/ N leader and C tail + his tag
GVSDVPRDLEVVAATPTSLLISWTSVLLKDYRITYGETGGNSPVQEFTVPDQHATISGLKPGVDYTITVYALQNAHHERLYISINYRTEIDKPSQHHHHHH

SEQ ID NO: 318 - protein, 90 aa, Artificial Sequence
  Synthetic: ATI_1421_H05 w/ N leader and modified C-terminus including PC
GVSDVPRDLEVVAATPTSLLISWTSVLLKDYRITYGETGGNSPVQEFTVPDQHATISGLKPGVDYTITVYALQNAHHERLYISINYRTPC

SEQ ID NO: 319 - protein, 96 aa, Artificial Sequence
  Synthetic: ATI_1421_H05 w/ N leader and modified C-terminus including PC + his tag
GVSDVPRDLEVVAATPTSLLISWTSVLLKDYRITYGETGGNSPVQEFTVPDQHATISGLKPGVDYTITVYALQNAHHERLYISINYRTPCHHHHHH

SEQ ID NO: 320 - protein, 102 aa, Artificial Sequence
  Synthetic: ATI_1421_H05 full length
MGVSDVPRDLEVVAATPTSLLISWTSVLLKDYRITYGETGGNSPVQEFTVPDQHATISGLKPGVDYTITVYALQNAHHERLYISINYRTEIDKPSQHHHHHH

SEQ ID NO: 321 - protein, 79 aa, Artificial Sequence
  Synthetic: ATI_1422_E06 core
EVVAATPTSLLISWLPSYYITYRITYGETGGNSPVQEFTVSKDLATISGLKPGVDYTITVYAFNGSSYYTFGISINYRT

SEQ ID NO: 322 - protein, 7 aa, Artificial Sequence
  Synthetic: ATI_1422_E06 BC loop
LPSYYIT

SEQ ID NO: 323 - protein, 4 aa, Artificial Sequence
  Synthetic: ATI_1422_E06 DE loop
SKDL

SEQ ID NO: 324 - protein, 10 aa, Artificial Sequence
  Synthetic: ATI_1422_E06 FG loop
FNGSSYYTFG

SEQ ID NO: 325 - protein, 88 aa, Artificial Sequence
  Synthetic: ATI_1422_E06 w/ N leader
GVSDVPRDLEVVAATPTSLLISWLPSYYITYRITYGETGGNSPVQEFTVSKDLATISGLKPGVDYTITVYAFNGSSYYTFGISINYRT

SEQ ID NO: 326 - protein, 101 aa, Artificial Sequence
  Synthetic: ATI_1422_E06 w/ N leader + his tag
GVSDVPRDLEVVAATPTSLLISWLPSYYITYRITYGETGGNSPVQEFTVSKDLATISGLKPGVDYTITVYAFNGSSYYTFGISINYRTEIDKPSQHHHHHH

SEQ ID NO: 327 - protein, 101 aa, Artificial Sequence; identical to SEQ ID NO: 326
  Synthetic: ATI_1422_E06 w/ N leader and C tail

SEQ ID NO: 328 - protein, 90 aa, Artificial Sequence
  Synthetic: ATI_1422_E06 w/ N leader and C tail + his tag
GVSDVPRDLEVVAATPTSLLISWLPSYYITYRITYGETGGNSPVQEFTVSKDLATISGLKPGVDYTITVYAFNGSSYYTFGISINYRTPC

SEQ ID NO: 329 - protein, 96 aa, Artificial Sequence
  Synthetic: ATI_1422_E06 w/ N leader and modified C-terminus including PC
GVSDVPRDLEVVAATPTSLLISWLPSYYITYRITYGETGGNSPVQEFTVSKDLATISGLKPGVDYTITVYAFNGSSYYTFGISINYRTPCHHHHHH

SEQ ID NO: 330 - protein, 101 aa, Artificial Sequence; identical to SEQ ID NO: 326
  Synthetic: ATI_1422_E06 w/ N leader and modified C-terminus including PC + his tag

SEQ ID NO: 331 - protein, 89 aa, Artificial Sequence
  Synthetic: ATI_1422_E06 full length
MGVSDVPRDLEVVAATPTSLLISWLPSYYITYRITYGETGGNSPVQEFTVSKDLATISGLKPGVDYTITVYAFNGSSYYTFGISINYRT

SEQ ID NO: 332 - protein, 78 aa, Artificial Sequence
  Synthetic: ATI_1422_F04 core
EVVAATPTSLLISWSIPSYFISYRITYGETGGNSPVQEFTVYKNYATISGLKPGVDYTITVYASEGIMFYNISINYRT

SEQ ID NO: 333 - protein, 8 aa, Artificial Sequence
  Synthetic: ATI_1422_F04 BC loop
SIPSYFIS

SEQ ID NO: 334 - protein, 4 aa, Artificial Sequence
  Synthetic: ATI_1422_F04 DE loop
YKNY

SEQ ID NO: 335 - protein, 8 aa, Artificial Sequence
  Synthetic: ATI_1422_F04 FG loop
SEGIMFYN

SEQ ID NO: 336 - protein, 87 aa, Artificial Sequence
  Synthetic: ATI_1422_F04w/ N leader
GVSDVPRDLEVVAATPTSLLISWSIPSYFISYRITYGETGGNSPVQEFTVYKNYATISGLKPGVDYTITVYASEGIMFYNISINYRT

SEQ ID NO: 337 - protein, 93 aa, Artificial Sequence
  Synthetic: ATI_1422_F04w/ N leader + his tag
GVSDVPRDLEVVAATPTSLLISWSIPSYFISYRITYGETGGNSPVQEFTVYKNYATISGLKPGVDYTITVYASEGIMFYNISINYRTHHHHHH

SEQ ID NO: 338 - protein, 94 aa, Artificial Sequence
  Synthetic: ATI_1422_F04 w/ N leader and C tail
GVSDVPRDLEVVAATPTSLLISWSIPSYFISYRITYGETGGNSPVQEFTVYKNYATISGLKPGVDYTITVYASEGIMFYNISINYRTEIDKPSQ

SEQ ID NO: 339 - protein, 100 aa, Artificial Sequence
  Synthetic: ATI_1422_F04 w/ N leader and C tail + his tag
GVSDVPRDLEVVAATPTSLLISWSIPSYFISYRITYGETGGNSPVQEFTVYKNYATISGLKPGVDYTITVYASEGIMFYNISINYRTEIDKPSQHHHHHH

SEQ ID NO: 340 - protein, 89 aa, Artificial Sequence
  Synthetic: ATI_1422_F04 w/ N leader and modified C-terminus including PC
GVSDVPRDLEVVAATPTSLLISWSIPSYFISYRITYGETGGNSPVQEFTVYKNYATISGLKPGVDYTITVYASEGIMFYNISINYRTPC

SEQ ID NO: 341 - protein, 95 aa, Artificial Sequence
  Synthetic: ATI_1422_F04 w/ N leader and modified C-terminus including PC + his tag
GVSDVPRDLEVVAATPTSLLISWSIPSYFISYRITYGETGGNSPVQEFTVYKNYATISGLKPGVDYTITVYASEGIMFYNISINYRTPCHHHHHH

SEQ ID NO: 342 - protein, 101 aa, Artificial Sequence
  Synthetic: ATI_1422_F04 full length
MGVSDVPRDLEVVAATPTSLLISWSIPSYFISYRITYGETGGNSPVQEFTVYKNYATISGLKPGVDYTITVYASEGIMFYNISINYRTEIDKPSQHHHHHH

SEQ ID NO: 343 - protein, 77 aa, Artificial Sequence
  Synthetic: ATI_1422_F05 core
EVVAATPTSLLISWPYPRGPYVFYRITYGETGGNSPVQEFTVYPGQATISGLKPGVDYTITVYAYTSGYVISINYRT

SEQ ID NO: 344 - protein, 9 aa, Artificial Sequence
  Synthetic: ATI_1422_F05 BC loop
PYPRGPYVF

SEQ ID NO: 345 - protein, 4 aa, Artificial Sequence
  Synthetic: ATI_1422_F05 DE loop
YPGQ

SEQ ID NO: 346 - protein, 6 aa, Artificial Sequence
  Synthetic: ATI_1422_F05 FG loop
YTSGYV

SEQ ID NO: 347 - protein, 86 aa, Artificial Sequence
  Synthetic: ATI_1422_F05 w/ N leader
GVSDVPRDLEVVAATPTSLLISWPYPRGPYVFYRITYGETGGNSPVQEFTVYPGQATISGLKPGVDYTITVYAYTSGYVISINYRT

SEQ ID NO: 348 - protein, 99 aa, Artificial Sequence
  Synthetic: ATI_1422_F05 w/ N leader + his tag
GVSDVPRDLEVVAATPTSLLISWPYPRGPYVFYRITYGETGGNSPVQEFTVYPGQATISGLKPGVDYTITVYAYTSGYVISINYRTEIDKPSQHHHHHH

SEQ ID NO: 349 - protein, 93 aa, Artificial Sequence
  Synthetic: ATI_1422_F05 w/ N leader and C tail
GVSDVPRDLEVVAATPTSLLISWPYPRGPYVFYRITYGETGGNSPVQEFTVYPGQATISGLKPGVDYTITVYAYTSGYVISINYRTEIDKPSQ

SEQ ID NO: 350 - protein, 99 aa, Artificial Sequence; identical to SEQ ID NO: 348
  Synthetic: ATI_1422_F05 w/ N leader and C tail + his tag

SEQ ID NO: 351 - protein, 88 aa, Artificial Sequence
  Synthetic: ATI_1422_F05 w/ N leader and modified C-terminus including PC
GVSDVPRDLEVVAATPTSLLISWPYPRGPYVFYRITYGETGGNSPVQEFTVYPGQATISGLKPGVDYTITVYAYTSGYVISINYRTPC

SEQ ID NO: 352 - protein, 94 aa, Artificial Sequence
  Synthetic: ATI_1422_F05 w/ N leader and modified C-terminus including PC + his tag
GVSDVPRDLEVVAATPTSLLISWPYPRGPYVFYRITYGETGGNSPVQEFTVYPGQATISGLKPGVDYTITVYAYTSGYVISINYRTPCHHHHHH

SEQ ID NO: 353 - protein, 100 aa, Artificial Sequence
  Synthetic: ATI_1422_F05 full length
MGVSDVPRDLEVVAATPTSLLISWPYPRGPYVFYRITYGETGGNSPVQEFTVYPGQATISGLKPGVDYTITVYAYTSGYVISINYRTEIDKPSQHHHHHH

SEQ ID NO: 354 - protein, 80 aa, Artificial Sequence
  Synthetic: ATI_1422_H04 core
EVVAATPTSLLISWYLPSYYVQYRITYGETGGNSPVQEFTVKSYNATISGLKPGVDYTITVYARMGVYYLSYSISINYRT

SEQ ID NO: 355 - protein, 8 aa, Artificial Sequence
  Synthetic: ATI_1422_H04 BC loop
YLPSYYVQ

SEQ ID NO: 356 - protein, 4 aa, Artificial Sequence
  Synthetic: ATI_1422_H04 DE loop
KSYN

SEQ ID NO: 357 - protein, 10 aa, Artificial Sequence
  Synthetic: ATI_1422_H04 FG loop
RMGVYYLSYS

SEQ ID NO: 358 - protein, 89 aa, Artificial Sequence
  Synthetic: ATI_1422_H04 w/ N leader
GVSDVPRDLEVVAATPTSLLISWYLPSYYVQYRITYGETGGNSPVQEFTVKSYNATISGLKPGVDYTITVYARMGVYYLSYSISINYRT

SEQ ID NO: 359 - protein, 95 aa, Artificial Sequence
  Synthetic: ATI_1422_H04 w/ N leader + his tag
GVSDVPRDLEVVAATPTSLLISWYLPSYYVQYRITYGETGGNSPVQEFTVKSYNATISGLKPGVDYTITVYARMGVYYLSYSISINYRTHHHHHH

SEQ ID NO: 360 - protein, 96 aa, Artificial Sequence
  Synthetic: ATI_1422_H04 w/ N leader and C tail
GVSDVPRDLEVVAATPTSLLISWYLPSYYVQYRITYGETGGNSPVQEFTVKSYNATISGLKPGVDYTITVYARMGVYYLSYSISINYRTEIDKPSQ

SEQ ID NO: 361 - protein, 102 aa, Artificial Sequence
  Synthetic: ATI_1422_H04 w/ N leader and C tail + his tag
GVSDVPRDLEVVAATPTSLLISWYLPSYYVQYRITYGETGGNSPVQEFTVKSYNATISGLKPGVDYTITVYARMGVYYLSYSISINYRTEIDKPSQHHHHHH

SEQ ID NO: 362 - protein, 91 aa, Artificial Sequence
  Synthetic: ATI_1422_H04 w/ N leader and modified C-terminus including PC
GVSDVPRDLEVVAATPTSLLISWYLPSYYVQYRITYGETGGNSPVQEFTVKSYNATISGLKPGVDYTITVYARMGVYYLSYSISINYRTPC

SEQ ID NO: 363 - protein, 97 aa, Artificial Sequence
  Synthetic: ATI_1422_H04 w/ N leader and modified C-terminus including PC + his tag
GVSDVPRDLEVVAATPTSLLISWYLPSYYVQYRITYGETGGNSPVQEFTVKSYNATISGLKPGVDYTITVYARMGVYYLSYSISINYRTPCHHHHHH

SEQ ID NO: 364 - protein, 103 aa, Artificial Sequence
  Synthetic: ATI_1422_H04  full length
MGVSDVPRDLEVVAATPTSLLISWYLPSYYVQYRITYGETGGNSPVQEFTVKSYNATISGLKPGVDYTITVYARMGVYYLSYSISINYRTEIDKPSQHHHHHH

SEQ ID NO: 365 - protein, 78 aa, Artificial Sequence
  Synthetic: ATI_1422_H05 core
EVVAATPTSLLISWQGQLSPSFYRITYGETGGNSPVQEFTVVAGMATISGLKPGVDYTITVYATSDVYFYSISINYRT

SEQ ID NO: 366 - protein, 8 aa, Artificial Sequence
  Synthetic: ATI_1422_H05 BC loop
QGQLSPSF

SEQ ID NO: 367 - protein, 4 aa, Artificial Sequence
  Synthetic: ATI_1422_H05 DE loop
VAGM

SEQ ID NO: 368 - protein, 8 aa, Artificial Sequence
  Synthetic: ATI_1422_H05 FG loop
TSDVYFYS

SEQ ID NO: 369 - protein, 87 aa, Artificial Sequence
  Synthetic: ATI_1422_H05 w/ N leader
GVSDVPRDLEVVAATPTSLLISWQGQLSPSFYRITYGETGGNSPVQEFTVVAGMATISGLKPGVDYTITVYATSDVYFYSISINYRT

SEQ ID NO: 370 - protein, 93 aa, Artificial Sequence
  Synthetic: ATI_1422_H05 w/ N leader + his tag
GVSDVPRDLEVVAATPTSLLISWQGQLSPSFYRITYGETGGNSPVQEFTVVAGMATISGLKPGVDYTITVYATSDVYFYSISINYRTHHHHHH

SEQ ID NO: 371 - protein, 94 aa, Artificial Sequence
  Synthetic: ATI_1422_H05 w/ N leader and C tail
GVSDVPRDLEVVAATPTSLLISWQGQLSPSFYRITYGETGGNSPVQEFTVVAGMATISGLKPGVDYTITVYATSDVYFYSISINYRTEIDKPSQ

SEQ ID NO: 372 - protein, 100 aa, Artificial Sequence
  Synthetic: ATI_1422_H05 w/ N leader and C tail + his tag
GVSDVPRDLEVVAATPTSLLISWQGQLSPSFYRITYGETGGNSPVQEFTVVAGMATISGLKPGVDYTITVYATSDVYFYSISINYRTEIDKPSQHHHHHH

SEQ ID NO: 373 - protein, 89 aa, Artificial Sequence
  Synthetic: ATI_1422_H05 w/ N leader and modified C-terminus including PC
GVSDVPRDLEVVAATPTSLLISWQGQLSPSFYRITYGETGGNSPVQEFTVVAGMATISGLKPGVDYTITVYATSDVYFYSISINYRTPC

SEQ ID NO: 374 - protein, 95 aa, Artificial Sequence
  Synthetic: ATI_1422_H05 w/ N leader and modified C-terminus including PC + his tag
GVSDVPRDLEVVAATPTSLLISWQGQLSPSFYRITYGETGGNSPVQEFTVVAGMATISGLKPGVDYTITVYATSDVYFYSISINYRTPCHHHHHH

SEQ ID NO: 375 - protein, 101 aa, Artificial Sequence
  Synthetic:  full length
MGVSDVPRDLEVVAATPTSLLISWQGQLSPSFYRITYGETGGNSPVQEFTVVAGMATISGLKPGVDYTITVYATSDVYFYSISINYRTEIDKPSQHHHHHH

SEQ ID NO: 376 - protein, 82 aa, Artificial Sequence
  Synthetic: ATI_1422_G05 core
EVVAATPTSLLISWIAPYYSVIYRITYGETGGNSPVQEFTVTGSGYATISGLKPGVDYTITVYATYCASVASYAFISINYRT

SEQ ID NO: 377 - protein, 8 aa, Artificial Sequence
  Synthetic: ATI_1422_G05 BC loop
IAPYYSVI

SEQ ID NO: 378 - protein, 5 aa, Artificial Sequence
  Synthetic: ATI_1422_G05 DE loop
TGSGY

SEQ ID NO: 379 - protein, 11 aa, Artificial Sequence
  Synthetic: ATI_1422_G05 FG loop
TYCASVASYAF

SEQ ID NO: 380 - protein, 91 aa, Artificial Sequence
  Synthetic: ATI_1422_G05 w/ N leader
GVSDVPRDLEVVAATPTSLLISWIAPYYSVIYRITYGETGGNSPVQEFTVTGSGYATISGLKPGVDYTITVYATYCASVASYAFISINYRT

SEQ ID NO: 381 - protein, 97 aa, Artificial Sequence
  Synthetic: ATI_1422_G05 w/ N leader + his tag
GVSDVPRDLEVVAATPTSLLISWIAPYYSVIYRITYGETGGNSPVQEFTVTGSGYATISGLKPGVDYTITVYATYCASVASYAFISINYRTHHHHHH

SEQ ID NO: 382 - protein, 98 aa, Artificial Sequence
  Synthetic: ATI_1422_G05 w/ N leader and C tail
GVSDVPRDLEVVAATPTSLLISWIAPYYSVIYRITYGETGGNSPVQEFTVTGSGYATISGLKPGVDYTITVYATYCASVASYAFISINYRTEIDKPSQ

SEQ ID NO: 383 - protein, 104 aa, Artificial Sequence
  Synthetic: ATI_1422_G05 w/ N leader and C tail + his tag
GVSDVPRDLEVVAATPTSLLISWIAPYYSVIYRITYGETGGNSPVQEFTVTGSGYATISGLKPGVDYTITVYATYCASVASYAFISINYRTEIDKPSQHHHHHH

SEQ ID NO: 384 - protein, 93 aa, Artificial Sequence
  Synthetic: ATI_1422_G05 w/ N leader and modified C-terminus including PC
GVSDVPRDLEVVAATPTSLLISWIAPYYSVIYRITYGETGGNSPVQEFTVTGSGYATISGLKPGVDYTITVYATYCASVASYAFISINYRTPC

SEQ ID NO: 385 - protein, 99 aa, Artificial Sequence
  Synthetic: ATI_1422_G05 w/ N leader and modified C-terminus including PC + his tag
GVSDVPRDLEVVAATPTSLLISWIAPYYSVIYRITYGETGGNSPVQEFTVTGSGYATISGLKPGVDYTITVYATYCASVASYAFISINYRTPCHHHHHH

SEQ ID NO: 386 - protein, 105 aa, Artificial Sequence
  Synthetic: ATI_1422_G05 full length
MGVSDVPRDLEVVAATPTSLLISWIAPYYSVIYRITYGETGGNSPVQEFTVTGSGYATISGLKPGVDYTITVYATYCASVASYAFISINYRTEIDKPSQHHHHHH

SEQ ID NO: 387 - protein, 82 aa, Artificial Sequence
  Synthetic: ATI_1760_C02 core
EVVAATPTSLLISWIAPYYSVIYRITYGETGGNSPVQEFTVPGSAYATISGLKPGVDYTITVYASSGASIAAYAFISINYRT

SEQ ID NO: 388 - protein, 8 aa, Artificial Sequence
  Synthetic: ATI_1760_C02 BC loop
IAPYYSVI

SEQ ID NO: 389 - protein, 5 aa, Artificial Sequence
  Synthetic: ATI_1760_C02 DE loop
PGSAY

SEQ ID NO: 390 - protein, 11 aa, Artificial Sequence
  Synthetic: ATI_1760_C02 FG loop
SSGASIAAYAF

SEQ ID NO: 391 - protein, 91 aa, Artificial Sequence
  Synthetic: ATI_1760_C02 w/ N leader
GVSDVPRDLEVVAATPTSLLISWIAPYYSVIYRITYGETGGNSPVQEFTVPGSAYATISGLKPGVDYTITVYASSGASIAAYAFISINYRT

SEQ ID NO: 392 - protein, 97 aa, Artificial Sequence
  Synthetic: ATI_1760_C02 w/ N leader + his tag
GVSDVPRDLEVVAATPTSLLISWIAPYYSVIYRITYGETGGNSPVQEFTVPGSAYATISGLKPGVDYTITVYASSGASIAAYAFISINYRTHHHHHH

SEQ ID NO: 393 - protein, 98 aa, Artificial Sequence
  Synthetic: ATI_1760_C02 w/ N leader and C tail
GVSDVPRDLEVVAATPTSLLISWIAPYYSVIYRITYGETGGNSPVQEFTVPGSAYATISGLKPGVDYTITVYASSGASIAAYAFISINYRTEIDKPSQ

SEQ ID NO: 394 - protein, 104 aa, Artificial Sequence
  Synthetic: ATI_1760_C02 w/ N leader and C tail + his tag
GVSDVPRDLEVVAATPTSLLISWIAPYYSVIYRITYGETGGNSPVQEFTVPGSAYATISGLKPGVDYTITVYASSGASIAAYAFISINYRTEIDKPSQHHHHHH

SEQ ID NO: 395 - protein, 93 aa, Artificial Sequence
  Synthetic: ATI_1760_C02 w/ N leader and modified C-terminus including PC
GVSDVPRDLEVVAATPTSLLISWIAPYYSVIYRITYGETGGNSPVQEFTVPGSAYATISGLKPGVDYTITVYASSGASIAAYAFISINYRTPC

SEQ ID NO: 396 - protein, 99 aa, Artificial Sequence
  Synthetic: ATI_1760_C02 w/ N leader and modified C-terminus including PC + his tag
GVSDVPRDLEVVAATPTSLLISWIAPYYSVIYRITYGETGGNSPVQEFTVPGSAYATISGLKPGVDYTITVYASSGASIAAYAFISINYRTPCHHHHHH

SEQ ID NO: 397 - protein, 105 aa, Artificial Sequence
  Synthetic: ATI_1760_C02 full length
MGVSDVPRDLEVVAATPTSLLISWIAPYYSVIYRITYGETGGNSPVQEFTVPGSAYATISGLKPGVDYTITVYASSGASIAAYAFISINYRTEIDKPSQHHHHHH

SEQ ID NO: 398 - protein, 82 aa, Artificial Sequence
  Synthetic: ATI_1760_E01 core
EVVAATPTSLLISWIAPYYSVKYRITYGETGGNSPVQEFTVAGADYATISGLKPGVDYTITVYATYGASIASYAFISINYRT

SEQ ID NO: 399 - protein, 8 aa, Artificial Sequence
  Synthetic: ATI_1760_E01 BC loop
IAPYYSVK

SEQ ID NO: 400 - protein, 5 aa, Artificial Sequence
  Synthetic: ATI_1760_E01 DE loop
AGADY

SEQ ID NO: 401 - protein, 11 aa, Artificial Sequence
  Synthetic: ATI_1760_E01 FG loop
TYGASIASYAF

SEQ ID NO: 402 - protein, 91 aa, Artificial Sequence
  Synthetic: ATI_1760_E01 w/ N leader
GVSDVPRDLEVVAATPTSLLISWIAPYYSVKYRITYGETGGNSPVQEFTVAGADYATISGLKPGVDYTITVYATYGASIASYAFISINYRT

SEQ ID NO: 403 - protein, 97 aa, Artificial Sequence
  Synthetic: ATI_1760_E01 w/ N leader + his tag
GVSDVPRDLEVVAATPTSLLISWIAPYYSVKYRITYGETGGNSPVQEFTVAGADYATISGLKPGVDYTITVYATYGASIASYAFISINYRTHHHHHH

SEQ ID NO: 404 - protein, 98 aa, Artificial Sequence
  Synthetic: ATI_1760_E01 w/ N leader and C tail
GVSDVPRDLEVVAATPTSLLISWIAPYYSVKYRITYGETGGNSPVQEFTVAGADYATISGLKPGVDYTITVYATYGASIASYAFISINYRTEIDKPSQ

SEQ ID NO: 405 - protein, 104 aa, Artificial Sequence
  Synthetic: ATI_1760_E01 w/ N leader and C tail + his tag
GVSDVPRDLEVVAATPTSLLISWIAPYYSVKYRITYGETGGNSPVQEFTVAGADYATISGLKPGVDYTITVYATYGASIASYAFISINYRTEIDKPSQHHHHHH

SEQ ID NO: 406 - protein, 93 aa, Artificial Sequence
  Synthetic: ATI_1760_E01 w/ N leader and modified C-terminus including PC
GVSDVPRDLEVVAATPTSLLISWIAPYYSVKYRITYGETGGNSPVQEFTVAGADYATISGLKPGVDYTITVYATYGASIASYAFISINYRTPC

SEQ ID NO: 407 - protein, 99 aa, Artificial Sequence
  Synthetic: ATI_1760_E01 w/ N leader and modified C-terminus including PC + his tag
GVSDVPRDLEVVAATPTSLLISWIAPYYSVKYRITYGETGGNSPVQEFTVAGADYATISGLKPGVDYTITVYATYGASIASYAFISINYRTPCHHHHHH

SEQ ID NO: 408 - protein, 105 aa, Artificial Sequence
  Synthetic: ATI_1760_E01 full length
MGVSDVPRDLEVVAATPTSLLISWIAPYYSVKYRITYGETGGNSPVQEFTVAGADYATISGLKPGVDYTITVYATYGASIASYAFISINYRTEIDKPSQHHHHHH

SEQ ID NO: 409 - protein, 82 aa, Artificial Sequence
  Synthetic: ATI_1760_F01 core
EVVAATPTSLLISWIAPYYAVMYRITYGETGGNSPVQEFTVPGGGYATISGLKPGVDYTITVYATGGASIAAYAFISINYRT

SEQ ID NO: 410 - protein, 8 aa, Artificial Sequence
  Synthetic: ATI_1760_F01 BC loop
IAPYYAVM

SEQ ID NO: 411 - protein, 5 aa, Artificial Sequence
  Synthetic: ATI_1760_F01 DE loop
PGGGY

SEQ ID NO: 412 - protein, 11 aa, Artificial Sequence
  Synthetic: ATI_1760_F01 FG loop
TGGASIAAYAF

SEQ ID NO: 413 - protein, 91 aa, Artificial Sequence
  Synthetic: ATI_1760_F01 w/ N leader
GVSDVPRDLEVVAATPTSLLISWIAPYYAVMYRITYGETGGNSPVQEFTVPGGGYATISGLKPGVDYTITVYATGGASIAAYAFISINYRT

SEQ ID NO: 414 - protein, 97 aa, Artificial Sequence
  Synthetic: ATI_1760_F01 w/ N leader + his tag
GVSDVPRDLEVVAATPTSLLISWIAPYYAVMYRITYGETGGNSPVQEFTVPGGGYATISGLKPGVDYTITVYATGGASIAAYAFISINYRTHHHHHH

SEQ ID NO: 415 - protein, 98 aa, Artificial Sequence
  Synthetic: ATI_1760_F01 w/ N leader and C tail
GVSDVPRDLEVVAATPTSLLISWIAPYYAVMYRITYGETGGNSPVQEFTVPGGGYATISGLKPGVDYTITVYATGGASIAAYAFISINYRTEIDKPSQ

SEQ ID NO: 416 - protein, 104 aa, Artificial Sequence
  Synthetic: ATI_1760_F01 w/ N leader and C tail + his tag
GVSDVPRDLEVVAATPTSLLISWIAPYYAVMYRITYGETGGNSPVQEFTVPGGGYATISGLKPGVDYTITVYATGGASIAAYAFISINYRTEIDKPSQHHHHHH

SEQ ID NO: 417 - protein, 93 aa, Artificial Sequence
  Synthetic: ATI_1760_F01 w/ N leader and modified C-terminus including PC
GVSDVPRDLEVVAATPTSLLISWIAPYYAVMYRITYGETGGNSPVQEFTVPGGGYATISGLKPGVDYTITVYATGGASIAAYAFISINYRTPC

SEQ ID NO: 418 - protein, 99 aa, Artificial Sequence
  Synthetic: ATI_1760_F01 w/ N leader and modified C-terminus including PC + his tag
GVSDVPRDLEVVAATPTSLLISWIAPYYAVMYRITYGETGGNSPVQEFTVPGGGYATISGLKPGVDYTITVYATGGASIAAYAFISINYRTPCHHHHHH

SEQ ID NO: 419 - protein, 105 aa, Artificial Sequence
  Synthetic: ATI_1760_F01 full length
MGVSDVPRDLEVVAATPTSLLISWIAPYYAVMYRITYGETGGNSPVQEFTVPGGGYATISGLKPGVDYTITVYATGGASIAAYAFISINYRTEIDKPSQHHHHHH

SEQ ID NO: 420 - protein, 79 aa, Artificial Sequence
  Synthetic: ATI_1494_D03 core
EVVAATPTSLLISWSYPSYHLYRITYGETGGNSPVQEFTVHIDYATISGLKPGVDYTITVYAQSPPYDIYYEISINYRT

SEQ ID NO: 421 - protein, 7 aa, Artificial Sequence
  Synthetic: ATI_1494_D03 BC loop
SYPSYHL

SEQ ID NO: 422 - protein, 4 aa, Artificial Sequence
  Synthetic: ATI_1494_D03 DE loop
HIDY

SEQ ID NO: 423 - protein, 10 aa, Artificial Sequence
  Synthetic: ATI_1494_D03 FG loop
QSPPYDIYYE

SEQ ID NO: 424 - protein, 88 aa, Artificial Sequence
  Synthetic: ATI_1494_D03 w/ N leader
GVSDVPRDLEVVAATPTSLLISWSYPSYHLYRITYGETGGNSPVQEFTVHIDYATISGLKPGVDYTITVYAQSPPYDIYYEISINYRT

SEQ ID NO: 425 - protein, 94 aa, Artificial Sequence
  Synthetic: ATI_1494_D03 w/ N leader + his tag
GVSDVPRDLEVVAATPTSLLISWSYPSYHLYRITYGETGGNSPVQEFTVHIDYATISGLKPGVDYTITVYAQSPPYDIYYEISINYRTHHHHHH

SEQ ID NO: 426 - protein, 95 aa, Artificial Sequence
  Synthetic: ATI_1494_D03 w/ N leader and C tail
GVSDVPRDLEVVAATPTSLLISWSYPSYHLYRITYGETGGNSPVQEFTVHIDYATISGLKPGVDYTITVYAQSPPYDIYYEISINYRTEIDKPSQ

SEQ ID NO: 427 - protein, 101 aa, Artificial Sequence
  Synthetic: ATI_1494_D03 w/ N leader and C tail + his tag
GVSDVPRDLEVVAATPTSLLISWSYPSYHLYRITYGETGGNSPVQEFTVHIDYATISGLKPGVDYTITVYAQSPPYDIYYEISINYRTEIDKPSQHHHHHH

SEQ ID NO: 428 - protein, 90 aa, Artificial Sequence
  Synthetic: ATI_1494_D03 w/ N leader and modified C-terminus including PC
GVSDVPRDLEVVAATPTSLLISWSYPSYHLYRITYGETGGNSPVQEFTVHIDYATISGLKPGVDYTITVYAQSPPYDIYYEISINYRTPC

SEQ ID NO: 429 - protein, 96 aa, Artificial Sequence
  Synthetic: ATI_1494_D03 w/ N leader and modified C-terminus including PC + his tag
GVSDVPRDLEVVAATPTSLLISWSYPSYHLYRITYGETGGNSPVQEFTVHIDYATISGLKPGVDYTITVYAQSPPYDIYYEISINYRTPCHHHHHH

SEQ ID NO: 430 - protein, 102 aa, Artificial Sequence
  Synthetic: ATI_1494_D03 full length
MGVSDVPRDLEVVAATPTSLLISWSYPSYHLYRITYGETGGNSPVQEFTVHIDYATISGLKPGVDYTITVYAQSPPYDIYYEISINYRTEIDKPSQHHHHHH

SEQ ID NO: 431 - protein, 79 aa, Artificial Sequence
  Synthetic: ATI_1494_D04 core
EVVAATPTSLLISWMESSSNSYRITYGETGGNSPVQEFTVPDQLATISGLKPGVDYTITVYALANAHYMRVGISINYRT

SEQ ID NO: 432 - protein, 7 aa, Artificial Sequence
  Synthetic: ATI_1494_D04 BC loop
MESSSNS

SEQ ID NO: 433 - protein, 4 aa, Artificial Sequence
  Synthetic: ATI_1494_D04 DE loop
PDQL

SEQ ID NO: 434 - protein, 10 aa, Artificial Sequence
  Synthetic: ATI_1494_D04 FG loop
LANAHYMRVG

SEQ ID NO: 435 - protein, 88 aa, Artificial Sequence
  Synthetic: ATI_1494_D04 w/ N leader
GVSDVPRDLEVVAATPTSLLISWMESSSNSYRITYGETGGNSPVQEFTVPDQLATISGLKPGVDYTITVYALANAHYMRVGISINYRT

SEQ ID NO: 436 - protein, 94 aa, Artificial Sequence
  Synthetic: ATI_1494_D04 w/ N leader + his tag
GVSDVPRDLEVVAATPTSLLISWMESSSNSYRITYGETGGNSPVQEFTVPDQLATISGLKPGVDYTITVYALANAHYMRVGISINYRTHHHHHH

SEQ ID NO: 437 - protein, 95 aa, Artificial Sequence
  Synthetic: ATI_1494_D04 w/ N leader and C tail
GVSDVPRDLEVVAATPTSLLISWMESSSNSYRITYGETGGNSPVQEFTVPDQLATISGLKPGVDYTITVYALANAHYMRVGISINYRTEIDKPSQ

SEQ ID NO: 438 - protein, 101 aa, Artificial Sequence
  Synthetic: ATI_1494_D04 w/ N leader and C tail + his tag
GVSDVPRDLEVVAATPTSLLISWMESSSNSYRITYGETGGNSPVQEFTVPDQLATISGLKPGVDYTITVYALANAHYMRVGISINYRTEIDKPSQHHHHHH

SEQ ID NO: 439 - protein, 90 aa, Artificial Sequence
  Synthetic: ATI_1494_D04 w/ N leader and modified C-terminus including PC
GVSDVPRDLEVVAATPTSLLISWMESSSNSYRITYGETGGNSPVQEFTVPDQLATISGLKPGVDYTITVYALANAHYMRVGISINYRTPC

SEQ ID NO: 440 - protein, 96 aa, Artificial Sequence
  Synthetic: ATI_1494_D04 w/ N leader and modified C-terminus including PC + his tag
GVSDVPRDLEVVAATPTSLLISWMESSSNSYRITYGETGGNSPVQEFTVPDQLATISGLKPGVDYTITVYALANAHYMRVGISINYRTPCHHHHHH

SEQ ID NO: 441 - protein, 102 aa, Artificial Sequence
  Synthetic: ATI_1494_D04 full length
MGVSDVPRDLEVVAATPTSLLISWMESSSNSYRITYGETGGNSPVQEFTVPDQLATISGLKPGVDYTITVYALANAHYMRVGISINYRTEIDKPSQHHHHHH

SEQ ID NO: 442 - protein, 79 aa, Artificial Sequence
  Synthetic: ATI_1523_A08 core
  misc_feature (21)..(21): Xaa can be any naturally occurring amino acid
EVVAATPTSLLISWISVQTYXYRITYGETGGNSPVQEFTVPDQSATISGLKPGVDYTITVYALEKAHYYRQNISINYRT

SEQ ID NO: 443 - protein, 7 aa, Artificial Sequence
  Synthetic: ATI_1523_A08 BC loop
  misc_feature (7)..(7): Xaa can be any naturally occurring amino acid
ISVQTYX

SEQ ID NO: 444 - protein, 4 aa, Artificial Sequence
  Synthetic: ATI_1523_A08 DE loop
PDQS

SEQ ID NO: 445 - protein, 10 aa, Artificial Sequence
  Synthetic: ATI_1523_A08 FG loop
LEKAHYYRQN

SEQ ID NO: 446 - protein, 88 aa, Artificial Sequence
  Synthetic: ATI_1523_A08 w/ N leader
  misc_feature (30)..(30): Xaa can be any naturally occurring amino acid
GVSDVPRDLEVVAATPTSLLISWISVQTYXYRITYGETGGNSPVQEFTVPDQSATISGLKPGVDYTITVYALEKAHYYRQNISINYRT

SEQ ID NO: 447 - protein, 94 aa, Artificial Sequence
  Synthetic: ATI_1523_A08 w/ N leader + his tag
  misc_feature (30)..(30): Xaa can be any naturally occurring amino acid
GVSDVPRDLEVVAATPTSLLISWISVQTYXYRITYGETGGNSPVQEFTVPDQSATISGLKPGVDYTITVYALEKAHYYRQNISINYRTHHHHHH

SEQ ID NO: 448 - protein, 95 aa, Artificial Sequence
  Synthetic: ATI_1523_A08 w/ N leader and C tail
  misc_feature (30)..(30): Xaa can be any naturally occurring amino acid
GVSDVPRDLEVVAATPTSLLISWISVQTYXYRITYGETGGNSPVQEFTVPDQSATISGLKPGVDYTITVYALEKAHYYRQNISINYRTEIDKPSQ

SEQ ID NO: 449 - protein, 101 aa, Artificial Sequence
  Synthetic: ATI_1523_A08 w/ N leader and C tail + his tag
  misc_feature (30)..(30): Xaa can be any naturally occurring amino acid
GVSDVPRDLEVVAATPTSLLISWISVQTYXYRITYGETGGNSPVQEFTVPDQSATISGLKPGVDYTITVYALEKAHYYRQNISINYRTEIDKPSQHHHHHH

SEQ ID NO: 450 - protein, 90 aa, Artificial Sequence
  Synthetic: ATI_1523_A08 w/ N leader and modified C-terminus including PC
  misc_feature (30)..(30): Xaa can be any naturally occurring amino acid
GVSDVPRDLEVVAATPTSLLISWISVQTYXYRITYGETGGNSPVQEFTVPDQSATISGLKPGVDYTITVYALEKAHYYRQNISINYRTPC

SEQ ID NO: 451 - protein, 96 aa, Artificial Sequence
  Synthetic: ATI_1523_A08 w/ N leader and modified C-terminus including PC + his tag
  misc_feature (30)..(30): Xaa can be any naturally occurring amino acid
GVSDVPRDLEVVAATPTSLLISWISVQTYXYRITYGETGGNSPVQEFTVPDQSATISGLKPGVDYTITVYALEKAHYYRQNISINYRTPCHHHHHH

SEQ ID NO: 452 - protein, 102 aa, Artificial Sequence
  Synthetic: ATI_1523_A08 full length
  misc_feature (31)..(31): Xaa can be any naturally occurring amino acid
MGVSDVPRDLEVVAATPTSLLISWISVQTYXYRITYGETGGNSPVQEFTVPDQSATISGLKPGVDYTITVYALEKAHYYRQNISINYRTEIDKPSQHHHHHH

SEQ ID NO: 453 - protein, 79 aa, Artificial Sequence
  Synthetic: ATI_1523_B10 core
  misc_feature (20)..(20): Xaa can be any naturally occurring amino acid
EVVAATPTSLLISWVYHYDXQYRITYGETGGNSPVQEFTVPDQKATISGLKPGVDYTITVYALSEAHHKRDSISINYRT

SEQ ID NO: 454 - protein, 7 aa, Artificial Sequence
  Synthetic: ATI_1523_B10  BC loop
  misc_feature (6)..(6): Xaa can be any naturally occurring amino acid
VYHYDXQ

SEQ ID NO: 455 - protein, 4 aa, Artificial Sequence
  Synthetic: ATI_1523_B10  DE loop
PDQK

SEQ ID NO: 456 - protein, 10 aa, Artificial Sequence
  Synthetic: ATI_1523_B10  FG loop
LSEAHHKRDS

SEQ ID NO: 457 - protein, 88 aa, Artificial Sequence
  Synthetic: ATI_1523_B10 w/ N leader
  misc_feature (29)..(29): Xaa can be any naturally occurring amino acid
GVSDVPRDLEVVAATPTSLLISWVYHYDXQYRITYGETGGNSPVQEFTVPDQKATISGLKPGVDYTITVYALSEAHHKRDSISINYRT

SEQ ID NO: 458 - protein, 94 aa, Artificial Sequence
  Synthetic: ATI_1523_B10 w/ N leader + his tag
  misc_feature (29)..(29): Xaa can be any naturally occurring amino acid
GVSDVPRDLEVVAATPTSLLISWVYHYDXQYRITYGETGGNSPVQEFTVPDQKATISGLKPGVDYTITVYALSEAHHKRDSISINYRTHHHHHH

SEQ ID NO: 459 - protein, 95 aa, Artificial Sequence
  Synthetic: ATI_1523_B10 w/ N leader and C tail
  misc_feature (29)..(29): Xaa can be any naturally occurring amino acid
GVSDVPRDLEVVAATPTSLLISWVYHYDXQYRITYGETGGNSPVQEFTVPDQKATISGLKPGVDYTITVYALSEAHHKRDSISINYRTEIDKPSQ

SEQ ID NO: 460 - protein, 101 aa, Artificial Sequence
  Synthetic: ATI_1523_B10 w/ N leader and C tail + his tag
  misc_feature (29)..(29): Xaa can be any naturally occurring amino acid
GVSDVPRDLEVVAATPTSLLISWVYHYDXQYRITYGETGGNSPVQEFTVPDQKATISGLKPGVDYTITVYALSEAHHKRDSISINYRTEIDKPSQHHHHHH

SEQ ID NO: 461 - protein, 90 aa, Artificial Sequence
  Synthetic: ATI_1523_B10 w/ N leader and modified C-terminus including PC
  misc_feature (29)..(29): Xaa can be any naturally occurring amino acid
GVSDVPRDLEVVAATPTSLLISWVYHYDXQYRITYGETGGNSPVQEFTVPDQKATISGLKPGVDYTITVYALSEAHHKRDSISINYRTPC

SEQ ID NO: 462 - protein, 96 aa, Artificial Sequence
  Synthetic: ATI_1523_B10 w/ N leader and modified C-terminus including PC + his tag
  misc_feature (29)..(29): Xaa can be any naturally occurring amino acid
GVSDVPRDLEVVAATPTSLLISWVYHYDXQYRITYGETGGNSPVQEFTVPDQKATISGLKPGVDYTITVYALSEAHHKRDSISINYRTPCHHHHHH

SEQ ID NO: 463 - protein, 102 aa, Artificial Sequence
  Synthetic: ATI_1523_B10  full length
  misc_feature (30)..(30): Xaa can be any naturally occurring amino acid
MGVSDVPRDLEVVAATPTSLLISWVYHYDXQYRITYGETGGNSPVQEFTVPDQKATISGLKPGVDYTITVYALSEAHHKRDSISINYRTEIDKPSQHHHHHH

SEQ ID NO: 464 - protein, 79 aa, Artificial Sequence
  Synthetic: ATI_1523_C07 core
EVVAATPTSLLISWRMHTDPDYRITYGETGGNSPVQEFTVPDQEATISGLKPGVDYTITVYAIQTAHYYRINISINYRT

SEQ ID NO: 465 - protein, 7 aa, Artificial Sequence
  Synthetic: ATI_1523_C07 BC loop
RMHTDPD

SEQ ID NO: 466 - protein, 4 aa, Artificial Sequence
  Synthetic: ATI_1523_C07 DE loop
PDQE

SEQ ID NO: 467 - protein, 10 aa, Artificial Sequence
  Synthetic: ATI_1523_C07 FG loop
IQTAHYYRIN

SEQ ID NO: 468 - protein, 88 aa, Artificial Sequence
  Synthetic: ATI_1523_C07 w/ N leader
GVSDVPRDLEVVAATPTSLLISWRMHTDPDYRITYGETGGNSPVQEFTVPDQEATISGLKPGVDYTITVYAIQTAHYYRINISINYRT

SEQ ID NO: 469 - protein, 94 aa, Artificial Sequence
  Synthetic: ATI_1523_C07 w/ N leader + his tag
GVSDVPRDLEVVAATPTSLLISWRMHTDPDYRITYGETGGNSPVQEFTVPDQEATISGLKPGVDYTITVYAIQTAHYYRINISINYRTHHHHHH

SEQ ID NO: 470 - protein, 95 aa, Artificial Sequence
  Synthetic: ATI_1523_C07 w/ N leader and C tail
GVSDVPRDLEVVAATPTSLLISWRMHTDPDYRITYGETGGNSPVQEFTVPDQEATISGLKPGVDYTITVYAIQTAHYYRINISINYRTEIDKPSQ

SEQ ID NO: 471 - protein, 101 aa, Artificial Sequence
  Synthetic: ATI_1523_C07 w/ N leader and C tail + his tag
GVSDVPRDLEVVAATPTSLLISWRMHTDPDYRITYGETGGNSPVQEFTVPDQEATISGLKPGVDYTITVYAIQTAHYYRINISINYRTEIDKPSQHHHHHH

SEQ ID NO: 472 - protein, 90 aa, Artificial Sequence
  Synthetic: ATI_1523_C07 w/ N leader and modified C-terminus including PC
GVSDVPRDLEVVAATPTSLLISWRMHTDPDYRITYGETGGNSPVQEFTVPDQEATISGLKPGVDYTITVYAIQTAHYYRINISINYRTPC

SEQ ID NO: 473 - protein, 96 aa, Artificial Sequence
  Synthetic: ATI_1523_C07 w/ N leader and modified C-terminus including PC + his tag
GVSDVPRDLEVVAATPTSLLISWRMHTDPDYRITYGETGGNSPVQEFTVPDQEATISGLKPGVDYTITVYAIQTAHYYRINISINYRTPCHHHHHH

SEQ ID NO: 474 - protein, 102 aa, Artificial Sequence
  Synthetic: ATI_1523_C07 full length
MGVSDVPRDLEVVAATPTSLLISWRMHTDPDYRITYGETGGNSPVQEFTVPDQEATISGLKPGVDYTITVYAIQTAHYYRINISINYRTEIDKPSQHHHHHH

SEQ ID NO: 475 - protein, 79 aa, Artificial Sequence
  Synthetic: ATI_1523_D07 core
EVVAATPTSLLISWENLASYQYRITYGETGGNSPVQEFTVPDVQATISGLKPGVDYTITVYALPYIHMKQRVISINYRT

SEQ ID NO: 476 - protein, 7 aa, Artificial Sequence
  Synthetic: ATI_1523_D07 BC loop
ENLASYQ

SEQ ID NO: 477 - protein, 4 aa, Artificial Sequence
  Synthetic: ATI_1523_D07 DE loop
PDVQ

SEQ ID NO: 478 - protein, 10 aa, Artificial Sequence
  Synthetic: ATI_1523_D07 FG loop
LPYIHMKQRV

SEQ ID NO: 479 - protein, 88 aa, Artificial Sequence
  Synthetic: ATI_1523_D07 w/ N leader
GVSDVPRDLEVVAATPTSLLISWENLASYQYRITYGETGGNSPVQEFTVPDVQATISGLKPGVDYTITVYALPYIHMKQRVISINYRT

SEQ ID NO: 480 - protein, 94 aa, Artificial Sequence
  Synthetic: ATI_1523_D07 w/ N leader + his tag
GVSDVPRDLEVVAATPTSLLISWENLASYQYRITYGETGGNSPVQEFTVPDVQATISGLKPGVDYTITVYALPYIHMKQRVISINYRTHHHHHH

SEQ ID NO: 481 - protein, 95 aa, Artificial Sequence
  Synthetic: ATI_1523_D07 w/ N leader and C tail
GVSDVPRDLEVVAATPTSLLISWENLASYQYRITYGETGGNSPVQEFTVPDVQATISGLKPGVDYTITVYALPYIHMKQRVISINYRTEIDKPSQ

SEQ ID NO: 482 - protein, 101 aa, Artificial Sequence
  Synthetic: ATI_1523_D07 w/ N leader and C tail + his tag
GVSDVPRDLEVVAATPTSLLISWENLASYQYRITYGETGGNSPVQEFTVPDVQATISGLKPGVDYTITVYALPYIHMKQRVISINYRTEIDKPSQHHHHHH

SEQ ID NO: 483 - protein, 90 aa, Artificial Sequence
  Synthetic: ATI_1523_D07 w/ N leader and modified C-terminus including PC
GVSDVPRDLEVVAATPTSLLISWENLASYQYRITYGETGGNSPVQEFTVPDVQATISGLKPGVDYTITVYALPYIHMKQRVISINYRTPC

SEQ ID NO: 484 - protein, 96 aa, Artificial Sequence
  Synthetic: ATI_1523_D07 w/ N leader and modified C-terminus including PC + his tag
GVSDVPRDLEVVAATPTSLLISWENLASYQYRITYGETGGNSPVQEFTVPDVQATISGLKPGVDYTITVYALPYIHMKQRVISINYRTPCHHHHHH

SEQ ID NO: 485 - protein, 102 aa, Artificial Sequence
  Synthetic: ATI_1523_D07  full length
MGVSDVPRDLEVVAATPTSLLISWENLASYQYRITYGETGGNSPVQEFTVPDVQATISGLKPGVDYTITVYALPYIHMKQRVISINYRTEIDKPSQHHHHHH

SEQ ID NO: 486 - protein, 79 aa, Artificial Sequence
  Synthetic: ATI_1523_D08 core
EVVAATPTSLLISWMRYYDAYYRITYGETGGNSPVQEFTVPDQSATISGLKPGVDYTITVYALEKAHYYRQNISINYRT

SEQ ID NO: 487 - protein, 7 aa, Artificial Sequence
  Synthetic: ATI_1523_D08 BC loop
MRYYDAY

SEQ ID NO: 488 - protein, 4 aa, Artificial Sequence
  Synthetic: ATI_1523_D08 DE loop
PDQS

SEQ ID NO: 489 - protein, 10 aa, Artificial Sequence
  Synthetic: ATI_1523_D08 FG loop
LEKAHYYRQN

SEQ ID NO: 490 - protein, 88 aa, Artificial Sequence
  Synthetic: ATI_1523_D08 w/ N leader
GVSDVPRDLEVVAATPTSLLISWMRYYDAYYRITYGETGGNSPVQEFTVPDQSATISGLKPGVDYTITVYALEKAHYYRQNISINYRT

SEQ ID NO: 491 - protein, 94 aa, Artificial Sequence
  Synthetic: ATI_1523_D08 w/ N leader + his tag
GVSDVPRDLEVVAATPTSLLISWMRYYDAYYRITYGETGGNSPVQEFTVPDQSATISGLKPGVDYTITVYALEKAHYYRQNISINYRTHHHHHH

SEQ ID NO: 492 - protein, 95 aa, Artificial Sequence
  Synthetic: ATI_1523_D08 w/ N leader and C tail
GVSDVPRDLEVVAATPTSLLISWMRYYDAYYRITYGETGGNSPVQEFTVPDQSATISGLKPGVDYTITVYALEKAHYYRQNISINYRTEIDKPSQ

SEQ ID NO: 493 - protein, 101 aa, Artificial Sequence
  Synthetic: ATI_1523_D08 w/ N leader and C tail + his tag
GVSDVPRDLEVVAATPTSLLISWMRYYDAYYRITYGETGGNSPVQEFTVPDQSATISGLKPGVDYTITVYALEKAHYYRQNISINYRTEIDKPSQHHHHHH

SEQ ID NO: 494 - protein, 90 aa, Artificial Sequence
  Synthetic: ATI_1523_D08 w/ N leader and modified C-terminus including PC
GVSDVPRDLEVVAATPTSLLISWMRYYDAYYRITYGETGGNSPVQEFTVPDQSATISGLKPGVDYTITVYALEKAHYYRQNISINYRTPC

SEQ ID NO: 495 - protein, 96 aa, Artificial Sequence
  Synthetic: ATI_1523_D08 w/ N leader and modified C-terminus including PC + his tag
GVSDVPRDLEVVAATPTSLLISWMRYYDAYYRITYGETGGNSPVQEFTVPDQSATISGLKPGVDYTITVYALEKAHYYRQNISINYRTPCHHHHHH

SEQ ID NO: 496 - protein, 102 aa, Artificial Sequence
  Synthetic: ATI_1523_D08 full length
MGVSDVPRDLEVVAATPTSLLISWMRYYDAYYRITYGETGGNSPVQEFTVPDQSATISGLKPGVDYTITVYALEKAHYYRQNISINYRTEIDKPSQHHHHHH

SEQ ID NO: 497 - protein, 79 aa, Artificial Sequence
  Synthetic: ATI_1523_E08 core
EVVAATPTSLLISWHHYQHYEYRITYGETGGNSPVQEFTVPDMGATISGLKPGVDYTITVYALEEAHSDRSSISINYRT

SEQ ID NO: 498 - protein, 7 aa, Artificial Sequence
  Synthetic: ATI_1523_E08 BC loop
HHYQHYE

SEQ ID NO: 499 - protein, 4 aa, Artificial Sequence
  Synthetic: ATI_1523_E08 DE loop
PDMG

SEQ ID NO: 500 - protein, 10 aa, Artificial Sequence
  Synthetic: ATI_1523_E08  FG loop
LEEAHSDRSS

SEQ ID NO: 501 - protein, 88 aa, Artificial Sequence
  Synthetic: ATI_1523_E08 w/ N leader
GVSDVPRDLEVVAATPTSLLISWHHYQHYEYRITYGETGGNSPVQEFTVPDMGATISGLKPGVDYTITVYALEEAHSDRSSISINYRT

SEQ ID NO: 502 - protein, 94 aa, Artificial Sequence
  Synthetic: ATI_1523_E08 w/ N leader + his tag
GVSDVPRDLEVVAATPTSLLISWHHYQHYEYRITYGETGGNSPVQEFTVPDMGATISGLKPGVDYTITVYALEEAHSDRSSISINYRTHHHHHH

SEQ ID NO: 503 - protein, 95 aa, Artificial Sequence
  Synthetic: ATI_1523_E08 w/ N leader and C tail
GVSDVPRDLEVVAATPTSLLISWHHYQHYEYRITYGETGGNSPVQEFTVPDMGATISGLKPGVDYTITVYALEEAHSDRSSISINYRTEIDKPSQ

SEQ ID NO: 504 - protein, 101 aa, Artificial Sequence
  Synthetic: ATI_1523_E08 w/ N leader and C tail + his tag
GVSDVPRDLEVVAATPTSLLISWHHYQHYEYRITYGETGGNSPVQEFTVPDMGATISGLKPGVDYTITVYALEEAHSDRSSISINYRTEIDKPSQHHHHHH

SEQ ID NO: 505 - protein, 90 aa, Artificial Sequence
  Synthetic: ATI_1523_E08 w/ N leader and modified C-terminus including PC
GVSDVPRDLEVVAATPTSLLISWHHYQHYEYRITYGETGGNSPVQEFTVPDMGATISGLKPGVDYTITVYALEEAHSDRSSISINYRTPC

SEQ ID NO: 506 - protein, 96 aa, Artificial Sequence
  Synthetic: ATI_1523_E08 w/ N leader and modified C-terminus including PC + his tag
GVSDVPRDLEVVAATPTSLLISWHHYQHYEYRITYGETGGNSPVQEFTVPDMGATISGLKPGVDYTITVYALEEAHSDRSSISINYRTPCHHHHHH

SEQ ID NO: 507 - protein, 102 aa, Artificial Sequence
  Synthetic: ATI_1523_E08 full length
MGVSDVPRDLEVVAATPTSLLISWHHYQHYEYRITYGETGGNSPVQEFTVPDMGATISGLKPGVDYTITVYALEEAHSDRSSISINYRTEIDKPSQHHHHHH

SEQ ID NO: 508 - protein, 76 aa, Artificial Sequence
  Synthetic: ATI_1523_F01 core
EVVAATPTSLLISWYKPSTIVTYRITYGETGGNSPVQEFTVYGYNATISGLKPGVDYTITVYAVHGVRFISINYRT

SEQ ID NO: 509 - protein, 8 aa, Artificial Sequence
  Synthetic: ATI_1523_F01 BC loop
YKPSTIVT

SEQ ID NO: 510 - protein, 4 aa, Artificial Sequence
  Synthetic: ATI_1523_F01 DE loop
YGYN

SEQ ID NO: 511 - protein, 6 aa, Artificial Sequence
  Synthetic: ATI_1523_F01 FG loop
VHGVRF

SEQ ID NO: 512 - protein, 85 aa, Artificial Sequence
  Synthetic: ATI_1523_F01 w/ N leader
GVSDVPRDLEVVAATPTSLLISWYKPSTIVTYRITYGETGGNSPVQEFTVYGYNATISGLKPGVDYTITVYAVHGVRFISINYRT

SEQ ID NO: 513 - protein, 91 aa, Artificial Sequence
  Synthetic: ATI_1523_F01 w/ N leader + his tag
GVSDVPRDLEVVAATPTSLLISWYKPSTIVTYRITYGETGGNSPVQEFTVYGYNATISGLKPGVDYTITVYAVHGVRFISINYRTHHHHHH

SEQ ID NO: 514 - protein, 92 aa, Artificial Sequence
  Synthetic: ATI_1523_F01 w/ N leader and C tail
GVSDVPRDLEVVAATPTSLLISWYKPSTIVTYRITYGETGGNSPVQEFTVYGYNATISGLKPGVDYTITVYAVHGVRFISINYRTEIDKPSQ

SEQ ID NO: 515 - protein, 98 aa, Artificial Sequence
  Synthetic: ATI_1523_F01 w/ N leader and C tail + his tag
GVSDVPRDLEVVAATPTSLLISWYKPSTIVTYRITYGETGGNSPVQEFTVYGYNATISGLKPGVDYTITVYAVHGVRFISINYRTEIDKPSQHHHHHH

SEQ ID NO: 516 - protein, 87 aa, Artificial Sequence
  Synthetic: ATI_1523_F01 w/ N leader and modified C-terminus including PC
GVSDVPRDLEVVAATPTSLLISWYKPSTIVTYRITYGETGGNSPVQEFTVYGYNATISGLKPGVDYTITVYAVHGVRFISINYRTPC

SEQ ID NO: 517 - protein, 93 aa, Artificial Sequence
  Synthetic: ATI_1523_F01 w/ N leader and modified C-terminus including PC + his tag
GVSDVPRDLEVVAATPTSLLISWYKPSTIVTYRITYGETGGNSPVQEFTVYGYNATISGLKPGVDYTITVYAVHGVRFISINYRTPCHHHHHH

SEQ ID NO: 518 - protein, 99 aa, Artificial Sequence
  Synthetic: ATI_1523_F01 full length
MGVSDVPRDLEVVAATPTSLLISWYKPSTIVTYRITYGETGGNSPVQEFTVYGYNATISGLKPGVDYTITVYAVHGVRFISINYRTEIDKPSQHHHHHH

SEQ ID NO: 519 - protein, 78 aa, Artificial Sequence
  Synthetic: ATI_1523_F04 core
EVVAATPTSLLISWGGSLSPTFYRITYGETGGNSPVQEFTVTYQGATISGLKPGVDYTITVYATEGIVYYQISINYRT

SEQ ID NO: 520 - protein, 8 aa, Artificial Sequence
  Synthetic: ATI_1523_F04 BC loop
GGSLSPTF

SEQ ID NO: 521 - protein, 4 aa, Artificial Sequence
  Synthetic: ATI_1523_F04 DE loop
TYQG

SEQ ID NO: 522 - protein, 8 aa, Artificial Sequence
  Synthetic: ATI_1523_F04 FG loop
TEGIVYYQ

SEQ ID NO: 523 - protein, 87 aa, Artificial Sequence
  Synthetic: ATI_1523_F04 w/ N leader
GVSDVPRDLEVVAATPTSLLISWGGSLSPTFYRITYGETGGNSPVQEFTVTYQGATISGLKPGVDYTITVYATEGIVYYQISINYRT

SEQ ID NO: 524 - protein, 93 aa, Artificial Sequence
  Synthetic: ATI_1523_F04 w/ N leader + his tag
GVSDVPRDLEVVAATPTSLLISWGGSLSPTFYRITYGETGGNSPVQEFTVTYQGATISGLKPGVDYTITVYATEGIVYYQISINYRTHHHHHH

SEQ ID NO: 525 - protein, 94 aa, Artificial Sequence
  Synthetic: ATI_1523_F04 w/ N leader and C tail
GVSDVPRDLEVVAATPTSLLISWGGSLSPTFYRITYGETGGNSPVQEFTVTYQGATISGLKPGVDYTITVYATEGIVYYQISINYRTEIDKPSQ

SEQ ID NO: 526 - protein, 100 aa, Artificial Sequence
  Synthetic: ATI_1523_F04 w/ N leader and C tail + his tag
GVSDVPRDLEVVAATPTSLLISWGGSLSPTFYRITYGETGGNSPVQEFTVTYQGATISGLKPGVDYTITVYATEGIVYYQISINYRTEIDKPSQHHHHHH

SEQ ID NO: 527 - protein, 89 aa, Artificial Sequence
  Synthetic: ATI_1523_F04 w/ N leader and modified C-terminus including PC
GVSDVPRDLEVVAATPTSLLISWGGSLSPTFYRITYGETGGNSPVQEFTVTYQGATISGLKPGVDYTITVYATEGIVYYQISINYRTPC

SEQ ID NO: 528 - protein, 95 aa, Artificial Sequence
  Synthetic: ATI_1523_F04 w/ N leader and modified C-terminus including PC + his tag
GVSDVPRDLEVVAATPTSLLISWGGSLSPTFYRITYGETGGNSPVQEFTVTYQGATISGLKPGVDYTITVYATEGIVYYQISINYRTPCHHHHHH

SEQ ID NO: 529 - protein, 101 aa, Artificial Sequence
  Synthetic: ATI_1523_F04 full length
MGVSDVPRDLEVVAATPTSLLISWGGSLSPTFYRITYGETGGNSPVQEFTVTYQGATISGLKPGVDYTITVYATEGIVYYQISINYRTEIDKPSQHHHHHH

SEQ ID NO: 530 - protein, 79 aa, Artificial Sequence
  Synthetic: ATI_1523_F08 core
EVVAATPTSLLISWVYHYDAQYRITYGETGGNSPVQEFTVPDQKATISGLKPGVDYTITVYALPRAHMDRSHISINYRT

SEQ ID NO: 531 - protein, 7 aa, Artificial Sequence
  Synthetic: ATI_1523_F08 BC loop
VYHYDAQ

SEQ ID NO: 532 - protein, 4 aa, Artificial Sequence
  Synthetic: ATI_1523_F08 DE loop
PDQK

SEQ ID NO: 533 - protein, 10 aa, Artificial Sequence
  Synthetic: ATI_1523_F08 FG loop
LPRAHMDRSH

SEQ ID NO: 534 - protein, 88 aa, Artificial Sequence
  Synthetic: ATI_1523_F08 w/ N leader
GVSDVPRDLEVVAATPTSLLISWVYHYDAQYRITYGETGGNSPVQEFTVPDQKATISGLKPGVDYTITVYALPRAHMDRSHISINYRT

SEQ ID NO: 535 - protein, 94 aa, Artificial Sequence
  Synthetic: ATI_1523_F08 w/ N leader + his tag
GVSDVPRDLEVVAATPTSLLISWVYHYDAQYRITYGETGGNSPVQEFTVPDQKATISGLKPGVDYTITVYALPRAHMDRSHISINYRTHHHHHH

SEQ ID NO: 536 - protein, 95 aa, Artificial Sequence
  Synthetic: ATI_1523_F08 w/ N leader and C tail
GVSDVPRDLEVVAATPTSLLISWVYHYDAQYRITYGETGGNSPVQEFTVPDQKATISGLKPGVDYTITVYALPRAHMDRSHISINYRTEIDKPSQ

SEQ ID NO: 537 - protein, 101 aa, Artificial Sequence
  Synthetic: ATI_1523_F08 w/ N leader and C tail + his tag
GVSDVPRDLEVVAATPTSLLISWVYHYDAQYRITYGETGGNSPVQEFTVPDQKATISGLKPGVDYTITVYALPRAHMDRSHISINYRTEIDKPSQHHHHHH

SEQ ID NO: 538 - protein, 90 aa, Artificial Sequence
  Synthetic: ATI_1523_F08 w/ N leader and modified C-terminus including PC
GVSDVPRDLEVVAATPTSLLISWVYHYDAQYRITYGETGGNSPVQEFTVPDQKATISGLKPGVDYTITVYALPRAHMDRSHISINYRTPC

SEQ ID NO: 539 - protein, 96 aa, Artificial Sequence
  Synthetic: ATI_1523_F08 w/ N leader and modified C-terminus including PC + his tag
GVSDVPRDLEVVAATPTSLLISWVYHYDAQYRITYGETGGNSPVQEFTVPDQKATISGLKPGVDYTITVYALPRAHMDRSHISINYRTPCHHHHHH

SEQ ID NO: 540 - protein, 102 aa, Artificial Sequence
  Synthetic: ATI_1523_F08 full length
MGVSDVPRDLEVVAATPTSLLISWVYHYDAQYRITYGETGGNSPVQEFTVPDQKATISGLKPGVDYTITVYALPRAHMDRSHISINYRTEIDKPSQHHHHHH

SEQ ID NO: 541 - protein, 79 aa, Artificial Sequence
  Synthetic: ATI_1523_G06 core
EVVAATPTSLLISWRIKSYHKYRITYGETGGNSPVQEFTVRSYAATISGLKPGVDYTITVYAIMEETHLAYAISINYRT

SEQ ID NO: 542 - protein, 7 aa, Artificial Sequence
  Synthetic: ATI_1523_G06 BC loop
RIKSYHK

SEQ ID NO: 543 - protein, 4 aa, Artificial Sequence
  Synthetic: ATI_1523_G06 DE loop
RSYA

SEQ ID NO: 544 - protein, 10 aa, Artificial Sequence
  Synthetic: ATI_1523_G06 FG loop
IMEETHLAYA

SEQ ID NO: 545 - protein, 88 aa, Artificial Sequence
  Synthetic: ATI_1523_G06 w/ N leader
GVSDVPRDLEVVAATPTSLLISWRIKSYHKYRITYGETGGNSPVQEFTVRSYAATISGLKPGVDYTITVYAIMEETHLAYAISINYRT

SEQ ID NO: 546 - protein, 94 aa, Artificial Sequence
  Synthetic: ATI_1523_G06 w/ N leader + his tag
GVSDVPRDLEVVAATPTSLLISWRIKSYHKYRITYGETGGNSPVQEFTVRSYAATISGLKPGVDYTITVYAIMEETHLAYAISINYRTHHHHHH

SEQ ID NO: 547 - protein, 95 aa, Artificial Sequence
  Synthetic: ATI_1523_G06 w/ N leader and C tail
GVSDVPRDLEVVAATPTSLLISWRIKSYHKYRITYGETGGNSPVQEFTVRSYAATISGLKPGVDYTITVYAIMEETHLAYAISINYRTEIDKPSQ

SEQ ID NO: 548 - protein, 101 aa, Artificial Sequence
  Synthetic: ATI_1523_G06 w/ N leader and C tail + his tag
GVSDVPRDLEVVAATPTSLLISWRIKSYHKYRITYGETGGNSPVQEFTVRSYAATISGLKPGVDYTITVYAIMEETHLAYAISINYRTEIDKPSQHHHHHH

SEQ ID NO: 549 - protein, 90 aa, Artificial Sequence
  Synthetic: ATI_1523_G06 w/ N leader and modified C-terminus including PC
GVSDVPRDLEVVAATPTSLLISWRIKSYHKYRITYGETGGNSPVQEFTVRSYAATISGLKPGVDYTITVYAIMEETHLAYAISINYRTPC

SEQ ID NO: 550 - protein, 96 aa, Artificial Sequence
  Synthetic: ATI_1523_G06 w/ N leader and modified C-terminus including PC + his tag
GVSDVPRDLEVVAATPTSLLISWRIKSYHKYRITYGETGGNSPVQEFTVRSYAATISGLKPGVDYTITVYAIMEETHLAYAISINYRTPCHHHHHH

SEQ ID NO: 551 - protein, 102 aa, Artificial Sequence
  Synthetic: ATI_1523_G06 full length
MGVSDVPRDLEVVAATPTSLLISWRIKSYHKYRITYGETGGNSPVQEFTVRSYAATISGLKPGVDYTITVYAIMEETHLAYAISINYRTEIDKPSQHHHHHH

SEQ ID NO: 552 - protein, 79 aa, Artificial Sequence
  Synthetic: ATI_1523_G07 core
EVVAATPTSLLISWVYPQADDYRITYGETGGNSPVQEFTVPDQNATISGLKPGVDYTITVYALAEAHLVRIYISINYRT

SEQ ID NO: 553 - protein, 7 aa, Artificial Sequence
  Synthetic: ATI_1523_G07 BC loop
VYPQADD

SEQ ID NO: 554 - protein, 4 aa, Artificial Sequence
  Synthetic: ATI_1523_G07 DE loop
PDQN

SEQ ID NO: 555 - protein, 10 aa, Artificial Sequence
  Synthetic: ATI_1523_G07 FG loop
LAEAHLVRIY

SEQ ID NO: 556 - protein, 88 aa, Artificial Sequence
  Synthetic: ATI_1523_G07 w/ N leader
GVSDVPRDLEVVAATPTSLLISWVYPQADDYRITYGETGGNSPVQEFTVPDQNATISGLKPGVDYTITVYALAEAHLVRIYISINYRT

SEQ ID NO: 557 - protein, 94 aa, Artificial Sequence
  Synthetic: ATI_1523_G07 w/ N leader + his tag
GVSDVPRDLEVVAATPTSLLISWVYPQADDYRITYGETGGNSPVQEFTVPDQNATISGLKPGVDYTITVYALAEAHLVRIYISINYRTHHHHHH

SEQ ID NO: 558 - protein, 95 aa, Artificial Sequence
  Synthetic: ATI_1523_G07 w/ N leader and C tail
GVSDVPRDLEVVAATPTSLLISWVYPQADDYRITYGETGGNSPVQEFTVPDQNATISGLKPGVDYTITVYALAEAHLVRIYISINYRTEIDKPSQ

SEQ ID NO: 559 - protein, 101 aa, Artificial Sequence
  Synthetic: ATI_1523_G07 w/ N leader and C tail + his tag
GVSDVPRDLEVVAATPTSLLISWVYPQADDYRITYGETGGNSPVQEFTVPDQNATISGLKPGVDYTITVYALAEAHLVRIYISINYRTEIDKPSQHHHHHH

SEQ ID NO: 560 - protein, 90 aa, Artificial Sequence
  Synthetic: ATI_1523_G07 w/ N leader and modified C-terminus including PC
GVSDVPRDLEVVAATPTSLLISWVYPQADDYRITYGETGGNSPVQEFTVPDQNATISGLKPGVDYTITVYALAEAHLVRIYISINYRTPC

SEQ ID NO: 561 - protein, 96 aa, Artificial Sequence
  Synthetic: ATI_1523_G07 w/ N leader and modified C-terminus including PC + his tag
GVSDVPRDLEVVAATPTSLLISWVYPQADDYRITYGETGGNSPVQEFTVPDQNATISGLKPGVDYTITVYALAEAHLVRIYISINYRTPCHHHHHH

SEQ ID NO: 562 - protein, 102 aa, Artificial Sequence
  Synthetic: ATI_1523_G07 full length
MGVSDVPRDLEVVAATPTSLLISWVYPQADDYRITYGETGGNSPVQEFTVPDQNATISGLKPGVDYTITVYALAEAHLVRIYISINYRTEIDKPSQHHHHHH

SEQ ID NO: 563 - protein, 79 aa, Artificial Sequence
  Synthetic: ATI_1523_H07 core
  misc_feature (21)..(21): Xaa can be any naturally occurring amino acid
EVVAATPTSLLISWVYHYDAXYRITYGETGGNSPVQEFTVPDQKATISGLKPGVDYTITVYALSEAHHKRDSISINYRT

SEQ ID NO: 564 - protein, 7 aa, Artificial Sequence
  Synthetic: ATI_1523_H07 BC loop
  misc_feature (7)..(7): Xaa can be any naturally occurring amino acid
VYHYDAX

SEQ ID NO: 565 - protein, 4 aa, Artificial Sequence
  Synthetic: ATI_1523_H07 DE loop
PDQK

SEQ ID NO: 566 - protein, 10 aa, Artificial Sequence
  Synthetic: ATI_1523_H07 FG loop
LSEAHHKRDS

SEQ ID NO: 567 - protein, 88 aa, Artificial Sequence
  Synthetic: ATI_1523_H07 w/ N leader
  misc_feature (30)..(30): Xaa can be any naturally occurring amino acid
GVSDVPRDLEVVAATPTSLLISWVYHYDAXYRITYGETGGNSPVQEFTVPDQKATISGLKPGVDYTITVYALSEAHHKRDSISINYRT

SEQ ID NO: 568 - protein, 94 aa, Artificial Sequence
  Synthetic: ATI_1523_H07 w/ N leader + his tag
  misc_feature (30)..(30): Xaa can be any naturally occurring amino acid
GVSDVPRDLEVVAATPTSLLISWVYHYDAXYRITYGETGGNSPVQEFTVPDQKATISGLKPGVDYTITVYALSEAHHKRDSISINYRTHHHHHH

SEQ ID NO: 569 - protein, 95 aa, Artificial Sequence
  Synthetic: ATI_1523_H07 w/ N leader and C tail
  misc_feature (30)..(30): Xaa can be any naturally occurring amino acid
GVSDVPRDLEVVAATPTSLLISWVYHYDAXYRITYGETGGNSPVQEFTVPDQKATISGLKPGVDYTITVYALSEAHHKRDSISINYRTEIDKPSQ

SEQ ID NO: 570 - protein, 101 aa, Artificial Sequence
  Synthetic: ATI_1523_H07 w/ N leader and C tail + his tag
  misc_feature (30)..(30): Xaa can be any naturally occurring amino acid
GVSDVPRDLEVVAATPTSLLISWVYHYDAXYRITYGETGGNSPVQEFTVPDQKATISGLKPGVDYTITVYALSEAHHKRDSISINYRTEIDKPSQHHHHHH

SEQ ID NO: 571 - protein, 90 aa, Artificial Sequence
  Synthetic: ATI_1523_H07 w/ N leader and modified C-terminus including PC
  misc_feature (30)..(30): Xaa can be any naturally occurring amino acid
GVSDVPRDLEVVAATPTSLLISWVYHYDAXYRITYGETGGNSPVQEFTVPDQKATISGLKPGVDYTITVYALSEAHHKRDSISINYRTPC

SEQ ID NO: 572 - protein, 96 aa, Artificial Sequence
  Synthetic: ATI_1523_H07 w/ N leader and modified C-terminus including PC + his tag
  misc_feature (30)..(30): Xaa can be any naturally occurring amino acid
GVSDVPRDLEVVAATPTSLLISWVYHYDAXYRITYGETGGNSPVQEFTVPDQKATISGLKPGVDYTITVYALSEAHHKRDSISINYRTPCHHHHHH

SEQ ID NO: 573 - protein, 101 aa, Artificial Sequence; identical to SEQ ID NO: 570
  Synthetic: ATI_1523_H07 full length
  misc_feature (30)..(30): Xaa can be any naturally occurring amino acid

SEQ ID NO: 574 - protein, 10 aa, Artificial Sequence
  Synthetic: N-terminal leader
MGVSDVPRDL

SEQ ID NO: 575 - protein, 9 aa, Artificial Sequence
  Synthetic: N-terminal leader
GVSDVPRDL

SEQ ID NO: 576 - protein, 9 aa, Artificial Sequence
  Synthetic: N-terminal leader
  misc_feature (1)..(2): Xaa may or may not be present; if one is present, Xaa is Met or Gly; if two are present, Xaa is Met-Gly
XXSDVPRDL

SEQ ID NO: 577 - protein, 8 aa, Artificial Sequence
  Synthetic: N-terminal leader
  misc_feature (1)..(2): Xaa may or may not be present; if one is present, Xaa is Met or Gly; if two are present, Xaa is Met-Gly
XXDVPRDL

SEQ ID NO: 578 - protein, 7 aa, Artificial Sequence
  Synthetic: N-terminal leader
  misc_feature (1)..(2): Xaa may or may not be present; if one is present, Xaa is Met or Gly; if two are present, Xaa is Met-Gly
XXVPRDL

SEQ ID NO: 579 - protein, 6 aa, Artificial Sequence
  Synthetic: N-terminal leader
  misc_feature (1)..(2): Xaa may or may not be present; if one is present, Xaa is Met or Gly; if two are present, Xaa is Met-Gly
XXPRDL

SEQ ID NO: 580 - protein, 5 aa, Artificial Sequence
  Synthetic: N-terminal leader
  misc_feature (1)..(2): Xaa may or may not be present; if one is present, Xaa is Met or Gly; if two are present, Xaa is Met-Gly
XXRDL

SEQ ID NO: 581 - protein, 4 aa, Artificial Sequence
  Synthetic: N-terminal leader
  misc_feature (1)..(2): Xaa may or may not be present; if one is present, Xaa is Met or Gly; if two are present, Xaa is Met-Gly
XXDL

SEQ ID NO: 582 - protein, 6 aa, Artificial Sequence
  Synthetic: N-terminal leader
MASTSG

SEQ ID NO: 583 - protein, 20 aa, Artificial Sequence
  Synthetic: N-terminal leader
METDTLLLWVLLLWVPGSTG

SEQ ID NO: 584 - protein, 4 aa, Artificial Sequence
  Synthetic: C-terminal tail
EIEK

SEQ ID NO: 585 - protein, 5 aa, Artificial Sequence
  Synthetic: C-terminal tail
EGSGC

SEQ ID NO: 586 - protein, 7 aa, Artificial Sequence
  Synthetic: C-terminal tail
EIEKPCQ

SEQ ID NO: 587 - protein, 7 aa, Artificial Sequence
  Synthetic: C-terminal tail
EIEKPSQ

SEQ ID NO: 588 - protein, 5 aa, Artificial Sequence
  Synthetic: C-terminal tail
EIEKP

SEQ ID NO: 589 - protein, 6 aa, Artificial Sequence
  Synthetic: C-terminal tail
EIEKPS

SEQ ID NO: 590 - protein, 6 aa, Artificial Sequence
  Synthetic: C-terminal tail
EIEKPC

SEQ ID NO: 591 - protein, 4 aa, Artificial Sequence
  Synthetic: C-terminal tail
EIDK

SEQ ID NO: 592 - protein, 7 aa, Artificial Sequence
  Synthetic: C-terminal tail
EIDKPCQ

SEQ ID NO: 593 - protein, 7 aa, Artificial Sequence
  Synthetic: C-terminal tail
EIDKPSQ

SEQ ID NO: 594 - protein, 7 aa, Artificial Sequence
  Synthetic: C-terminal tail
EIEPKSS

SEQ ID NO: 595 - protein, 6 aa, Artificial Sequence
  Synthetic: C-terminal tail
EIDKPC

SEQ ID NO: 596 - protein, 5 aa, Artificial Sequence
  Synthetic: C-terminal tail
EIDKP

SEQ ID NO: 597 - protein, 6 aa, Artificial Sequence
  Synthetic: C-terminal tail
EIDKPS

SEQ ID NO: 598 - protein, 9 aa, Artificial Sequence
  Synthetic: C-terminal tail
EIDKPSQLE

SEQ ID NO: 599 - protein, 12 aa, Artificial Sequence
  Synthetic: C-terminal tail
EIEDEDEDEDED

SEQ ID NO: 600 - protein, 5 aa, Artificial Sequence
  Synthetic: C-terminal tail
EGSGS

SEQ ID NO: 601 - protein, 9 aa, Artificial Sequence
  Synthetic: C-terminal tail
EIDKPCQLE

SEQ ID NO: 602 - protein, 13 aa, Artificial Sequence
  Synthetic: C-terminal tail
EIDKPSQHHHHHH

SEQ ID NO: 603 - protein, 10 aa, Artificial Sequence
  Synthetic: C-terminal tail
GSGCHHHHHH

SEQ ID NO: 604 - protein, 11 aa, Artificial Sequence
  Synthetic: C-terminal tail
EGSGCHHHHHH

SEQ ID NO: 605 - protein, 4 aa, Artificial Sequence
  Synthetic: C-terminal tail
PIDK

SEQ ID NO: 606 - protein, 4 aa, Artificial Sequence
  Synthetic: C-terminal tail
PIEK

SEQ ID NO: 607 - protein, 5 aa, Artificial Sequence
  Synthetic: C-terminal tail
PIDKP

SEQ ID NO: 608 - protein, 5 aa, Artificial Sequence
  Synthetic: C-terminal tail
PIEKP

SEQ ID NO: 609 - protein, 6 aa, Artificial Sequence
  Synthetic: C-terminal tail
PIDKPS

SEQ ID NO: 610 - protein, 6 aa, Artificial Sequence
  Synthetic: C-terminal tail
PIEKPS

SEQ ID NO: 611 - protein, 6 aa, Artificial Sequence
  Synthetic: C-terminal tail
PIDKPC

SEQ ID NO: 612 - protein, 6 aa, Artificial Sequence
  Synthetic: C-terminal tail
PIEKPC

SEQ ID NO: 613 - protein, 7 aa, Artificial Sequence
  Synthetic: C-terminal tail
PIDKPSQ

SEQ ID NO: 614 - protein, 7 aa, Artificial Sequence
  Synthetic: C-terminal tail
PIEKPSQ

SEQ ID NO: 615 - protein, 7 aa, Artificial Sequence
  Synthetic: C-terminal tail
PIDKPCQ

SEQ ID NO: 616 - protein, 7 aa, Artificial Sequence
  Synthetic: C-terminal tail
PIEKPCQ

SEQ ID NO: 617 - protein, 7 aa, Artificial Sequence
  Synthetic: C-terminal tail
PHHHHHH

SEQ ID NO: 618 - protein, 8 aa, Artificial Sequence
  Synthetic: C-terminal tail
PCHHHHHH

SEQ ID NO: 619 - protein, 6 aa, Artificial Sequence
  Synthetic: 6X-His tag
HHHHHH

SEQ ID NO: 620 - protein, 227 aa, Artificial Sequence
  Synthetic: Human IgG1 Fc domain
DKTHTCPPCPAPELLGGPSVFLFPPKPKDTLMISRTPEVTCVVVDVSHEDPEVKFNWYVDGVEVHNAKTKPREEQYNSTYRVVSVLTVLHQDWLNGKEYKCKVSNKALPAPIEKTISKAKGQPREPQVYTLPPSRDELTKNQVSLTCLVKGFYPSDIAVEWESNGQPENNYKTTPPVLDSDGSFFLYSKLTVDKSRWQQGNVFSCSVMHEALHNHYTQKSLSLSPGK

SEQ ID NO: 621 - protein, 16 aa, Artificial Sequence
  Synthetic: Core hinge region of Fc
DKTHTCPPCPAPELLG

SEQ ID NO: 622 - protein, 24 aa, Artificial Sequence
  Synthetic: Exemplary hinge sequence
EPKSSDKTHTCPPCPAPELLGGPS

SEQ ID NO: 623 - protein, 24 aa, Artificial Sequence
  Synthetic: Exemplary hinge sequence
EPKSSDKTHTCPPCPAPELLGGSS

SEQ ID NO: 624 - protein, 24 aa, Artificial Sequence
  Synthetic: Exemplary hinge sequence
EPKSSGSTHTCPPCPAPELLGGSS

SEQ ID NO: 625 - protein, 19 aa, Artificial Sequence
  Synthetic: Exemplary hinge sequence
DKTHTCPPCPAPELLGGPS

SEQ ID NO: 626 - protein, 19 aa, Artificial Sequence
  Synthetic: Exemplary hinge sequence
DKTHTCPPCPAPELLGGSS

SEQ ID NO: 627 - protein, 208 aa, Artificial Sequence
  Synthetic: Fc with CH2 and CH3 regions of IgG1 for Adnectin-hinge-Fc construct
VFLFPPKPKDTLMISRTPEVTCVVVDVSHEDPEVKFNWYVDGVEVHNAKTKPREEQYNSTYRVVSVLTVLHQDWLNGKEYKCKVSNKALPAPIEKTISKAKGQPREPQVYTLPPSRDELTKNQVSLTCLVKGFYPSDIAVEWESNGQPENNYKTTPPVLDSDGSFFLYSKLTVDKSRWQQGNVFSCSVMHEALHNHYTQKSLSLSPGK

SEQ ID NO: 628 - protein, 206 aa, Artificial Sequence
  Synthetic: Fc with CH2 and CH3 regions of IgG1 for Fc-hinge-Adnectin construct
VFLFPPKPKDTLMISRTPEVTCVVVDVSHEDPEVKFNWYVDGVEVHNAKTKPREEQYNSTYRVVSVLTVLHQDWLNGKEYKCKVSNKALPAPIEKTISKAKGQPREPQVYTLPPSRDELTKNQVSLTCLVKGFYPSDIAVEWESNGQPENNYKTTPPVLDSDGSFFLYSKLTVDKSRWQQGNVFSCSVMHEALHNHYTQKSLSLSP

SEQ ID NO: 629 - protein, 8 aa, Artificial Sequence
  Synthetic: Linker 1
GAGGGGSG

SEQ ID NO: 630 - protein, 6 aa, Artificial Sequence
  Synthetic: Linker 2
EPKSSD

SEQ ID NO: 631 - protein, 5 aa, Artificial Sequence
  Synthetic: Linker 3
PVGVV

SEQ ID NO: 632 - protein, 21 aa, Artificial Sequence
  Synthetic: Linker 4
ESPKAQASSVPTAQPQAEGLA

SEQ ID NO: 633 - protein, 17 aa, Artificial Sequence
  Synthetic: Linker 5
ELQLEESAAEAQDGELD

SEQ ID NO: 634 - protein, 9 aa, Artificial Sequence
  Synthetic: Linker 6
GQPDEPGGS

SEQ ID NO: 635 - protein, 13 aa, Artificial Sequence
  Synthetic: Linker 7
GGSGSGSGSGSGS

SEQ ID NO: 636 - protein, 17 aa, Artificial Sequence
  Synthetic: Linker 8
ELQLEESAAEAQEGELE

SEQ ID NO: 637 - protein, 5 aa, Artificial Sequence
  Synthetic: Linker 9
GSGSG

SEQ ID NO: 638 - protein, 4 aa, Artificial Sequence
  Synthetic: Linker 10
GSGC

SEQ ID NO: 639 - protein, 7 aa, Artificial Sequence
  Synthetic: Linker 11
AGGGGSG

SEQ ID NO: 640 - protein, 4 aa, Artificial Sequence
  Synthetic: Linker 12
GSGS

SEQ ID NO: 641 - protein, 8 aa, Artificial Sequence
  Synthetic: Linker 13
QPDEPGGS

SEQ ID NO: 642 - protein, 6 aa, Artificial Sequence
  Synthetic: Linker 14
GSGSGS

SEQ ID NO: 643 - protein, 6 aa, Artificial Sequence
  Synthetic: Linker 15
TVAAPS

SEQ ID NO: 644 - protein, 8 aa, Artificial Sequence
  Synthetic: Linker 16
KAGGGGSG

SEQ ID NO: 645 - protein, 13 aa, Artificial Sequence
  Synthetic: Linker 17
KGSGSGSGSGSGS

SEQ ID NO: 646 - protein, 9 aa, Artificial Sequence
  Synthetic: Linker 18
KQPDEPGGS

SEQ ID NO: 647 - protein, 18 aa, Artificial Sequence
  Synthetic: Linker 19
KELQLEESAAEAQDGELD

SEQ ID NO: 648 - protein, 7 aa, Artificial Sequence
  Synthetic: Linker 20
KTVAAPS

SEQ ID NO: 649 - protein, 9 aa, Artificial Sequence
  Synthetic: Linker 21
KAGGGGSGG

SEQ ID NO: 650 - protein, 14 aa, Artificial Sequence
  Synthetic: Linker 22
KGSGSGSGSGSGSG

SEQ ID NO: 651 - protein, 10 aa, Artificial Sequence
  Synthetic: Linker 23
KQPDEPGGSG

SEQ ID NO: 652 - protein, 19 aa, Artificial Sequence
  Synthetic: Linker 24
KELQLEESAAEAQDGELDG

SEQ ID NO: 653 - protein, 8 aa, Artificial Sequence
  Synthetic: Linker 25
KTVAAPSG

SEQ ID NO: 654 - protein, 8 aa, Artificial Sequence
  Synthetic: Linker 26
AGGGGSGG

SEQ ID NO: 655 - protein, 7 aa, Artificial Sequence
  Synthetic: Linker 27
AGGGGSG

SEQ ID NO: 656 - protein, 13 aa, Artificial Sequence
  Synthetic: Linker 28
GSGSGSGSGSGSG

SEQ ID NO: 657 - protein, 9 aa, Artificial Sequence
  Synthetic: Linker 29
QPDEPGGSG

SEQ ID NO: 658 - protein, 7 aa, Artificial Sequence
  Synthetic: Linker 30
TVAAPSG

SEQ ID NO: 659 - protein, 7 aa, Artificial Sequence
  Synthetic: Linker 31
PSTSTST

SEQ ID NO: 660 - protein, 7 aa, Artificial Sequence
  Synthetic: Linker 32
EIDKPSQ

SEQ ID NO: 661 - protein, 8 aa, Artificial Sequence
  Synthetic: Linker 33
GSGSGSGS

SEQ ID NO: 662 - protein, 10 aa, Artificial Sequence
  Synthetic: Linker 34
GSGSGSGSGS

SEQ ID NO: 663 - protein, 12 aa, Artificial Sequence
  Synthetic: Linker 35
GSGSGSGSGSGS

SEQ ID NO: 664 - protein, 14 aa, Artificial Sequence
  Synthetic: Linker 36
GSGSGSGSGSGSGS

SEQ ID NO: 665 - protein, 13 aa, Artificial Sequence
  Synthetic: Linker 37
GGSGSGSGSGSGS

SEQ ID NO: 666 - protein, 16 aa, Artificial Sequence
  Synthetic: Linker 38
GGSGSGSGSGSGSGSG

SEQ ID NO: 667 - protein, 15 aa, Artificial Sequence
  Synthetic: Linker 39
GSEGSEGSEGSEGSE

SEQ ID NO: 668 - protein, 8 aa, Artificial Sequence
  Synthetic: Linker 40
GGSEGGSE

SEQ ID NO: 669 - protein, 35 aa, Artificial Sequence
  Synthetic: Linker 41
GGGGSGGGGSGGGGSGGGGSGGGGSGGGGSGGGGS

SEQ ID NO: 670 - protein, 25 aa, Artificial Sequence
  Synthetic: Linker 42
GGGGSGGGGSGGGGSGGGGSGGGGS

SEQ ID NO: 671 - protein, 16 aa, Artificial Sequence
  Synthetic: Linker 43
GGGGSGGGGSGGGGSG

SEQ ID NO: 672 - protein, 7 aa, Artificial Sequence
  Synthetic: Linker 44
GPGPGPG

SEQ ID NO: 673 - protein, 11 aa, Artificial Sequence
  Synthetic: Linker 45
GPGPGPGPGPG

SEQ ID NO: 674 - protein, 6 aa, Artificial Sequence
  Synthetic: Linker 46
PAPAPA

SEQ ID NO: 675 - protein, 12 aa, Artificial Sequence
  Synthetic: Linker 47
PAPAPAPAPAPA

SEQ ID NO: 676 - protein, 18 aa, Artificial Sequence
  Synthetic: Linker 48
PAPAPAPAPAPAPAPAPA

SEQ ID NO: 677 - protein, 20 aa, Artificial Sequence
  Synthetic: Linker 49
GSGSGSGSGSGSGSGSGSGS

SEQ ID NO: 678 - protein, 20 aa, Artificial Sequence
  Synthetic: Linker 50
GGGGSGGGGSGGGGSGGGGS

SEQ ID NO: 679 - protein, 94 aa, Artificial Sequence
  Synthetic: ATI-968
VSDVPRDLEVVAATPTSLLISWIAPFYNVIYYRITYGETGGNSPVQEFTVPGTGYTATISGLKPGVDYTITVYAVTDGASIASYAFPISINYRT

SEQ ID NO: 680 - protein, 94 aa, Artificial Sequence
  Synthetic: ATI-964
VSDVPRDLEVVAATPTSLLISWSYDGSIERYYRITYGETGGNSPVQEFTVPPDQKTATISGLKPGVDYTITVYAVRLEEAHYYRESPISINYRT

SEQ ID NO: 681 - protein, 92 aa, Artificial Sequence
  Synthetic: ATI-967
VSDVPRDLEVVAATPTSLLISWQGQLSPSFYYRITYGETGGNSPVQEFTVPVASGTATISGLKPGVDYTITVYAVTSHGIYFYAPISINYRT

SEQ ID NO: 682 - protein, 94 aa, Artificial Sequence
  Synthetic: A02
VSDVPRDLEVVAATPTSLLISWSYDGPIDRYYRITYGETGGNSPVQEFTVPPDQKTATISGLKPGVDYTITVYAVRLEEAHYNREFPISINYRT

SEQ ID NO: 683 - protein, 92 aa, Artificial Sequence
  Synthetic: E01
VSDVPRDLEVVAATPTSLLISWRAQLSPSFYYRITYGETGGNSPVQEFTVPNDVMTATISGLKPGVDYTITVYAVTTHGVYFYSPISINYRT

SEQ ID NO: 684 - protein, 94 aa, Artificial Sequence
  Synthetic: ATI-965
VSDVPRDLEVVAATPTSLLISWTAYDSVDKYYRITYGETGGNSPVQEFTVGPRHHTATISGLKPGVDYTITVYAVYHTEPGYHAHMPISINYRT

SEQ ID NO: 685 - protein, 90 aa, Artificial Sequence
  Synthetic: ATI-966
VSDVPRDLEVVAATPTSLLISWHRFSSIMAYYRITYGETGGNSPVQEFTVAGSVNTATISGLKPGVDYTITVYAVTIHNVSFPISINYRT